European Patent Specification EP 4 244 342 B1, published April 1, 2026. Title: ENGINEERED MEGANUCLEASES HAVING SPECIFICITY FOR RECOGNITION SEQUENCES IN THE DYSTROPHIN GENE. Applicant: Precision BioSciences, Inc. Application Not Yet Assigned. The sequence listing filed with the application follows.

SEQUENCE LISTING (192 sequences)

SEQ ID NO: 1 - protein, 163 aa, Chlamydomonas reinhardtii
MNTKYNKEFLLYLAGFVDGDGSIIAQIKPNQSYKFKHQLSLAFQVTQKTQRRWFLDKLVDEIGVGYVRDRGSVSDYILSEIKPLHNFLTQLQPFLKLKQKQANLVLKIIWRLPSAKESPDKFLEVCTWVDQIAALNDSKTRKTTSETVRAVLDSLSEKKKSSP

SEQ ID NO: 2 - protein, 9 aa, Chlamydomonas reinhardtii
LAGLIDADG

SEQ ID NO: 3 - protein, 10 aa, Artificial Sequence
  Synthesized
MAPKKKRKVH

SEQ ID NO: 4 - protein, 3685 aa, Homo sapiens
MLWWEEVEDCYEREDVQKKTFTKWVNAQFSKFGKQHIENLFSDLQDGRRLLDLLEGLTGQKLPKEKGSTRVHALNNVNKALRVLQNNNVDLVNIGSTDIVDGNHKLTLGLIWNIILHWQVKNVMKNIMAGLQQTNSEKILLSWVRQSTRNYPQVNVINFTTSWSDGLALNALIHSHRPDLFDWNSVVCQQSATQRLEHAFNIARYQLGIEKLLDPEDVDTTYPDKKSILMYITSLFQVLPQQVSIEAIQEVEMLPRPPKVTKEEHFQLHHQMHYSQQITVSLAQGYERTSSPKPRFKSYAYTQAAYVTTSDPTRSPFPSQHLEAPEDKSFGSSLMESEVNLDRYQTALEEVLSWLLSAEDTLQAQGEISNDVEVVKDQFHTHEGYMMDLTAHQGRVGNILQLGSKLIGTGKLSEDEETEVQEQMNLLNSRWECLRVASMEKQSNLHRVLMDLQNQKLKELNDWLTKTEERTRKMEEEPLGPDLEDLKRQVQQHKVLQEDLEQEQVRVNSLTHMVVVVDESSGDHATAALEEQLKVLGDRWANICRWTEDRWVLLQDILLKWQRLTEEQCLFSAWLSEKEDAVNKIHTTGFKDQNEMLSSLQKLAVLKADLEKKKQSMGKLYSLKQDLLSTLKNKSVTQKTEAWLDNFARCWDNLVQKLEKSTAQISQAVTTTQPSLTQTTVMETVTTVTTREQILVKHAQEELPPPPPQKKRQITVDSEIRKRLDVDITELHSWITRSEAVLQSPEFAIFRKEGNFSDLKEKVNAIEREKAEKFRKLQDASRSAQALVEQMVNEGVNADSIKQASEQLNSRWIEFCQLLSERLNWLEYQNNIIAFYNQLQQLEQMTTTAENWLKIQPTTPSEPTAIKSQLKICKDEVNRLSDLQPQIERLKIQSIALKEKGQGPMFLDADFVAFTNHFKQVFSDVQAREKELQTIFDTLPPMRYQETMSAIRTWVQQSETKLSIPQLSVTDYEIMEQRLGELQALQSSLQEQQSGLYYLSTTVKEMSKKAPSEISRKYQSEFEEIEGRWKKLSSQLVEHCQKLEEQMNKLRKIQNHIQTLKKWMAEVDVFLKEEWPALGDSEILKKQLKQCRLLVSDIQTIQPSLNSVNEGGQKIKNEAEPEFASRLETELKELNTQWDHMCQQVYARKEALKGGLEKTVSLQKDLSEMHEWMTQAEEEYLERDFEYKTPDELQKAVEEMKRAKEEAQQKEAKVKLLTESVNSVIAQAPPVAQEALKKELETLTTNYQWLCTRLNGKCKTLEEVWACWHELLSYLEKANKWLNEVEFKLKTTENIPGGAEEISEVLDSLENLMRHSEDNPNQIRILAQTLTDGGVMDELINEELETFNSRWRELHEEAVRRQKLLEQSIQSAQETEKSLHLIQESLTFIDKQLAAYIADKVDAAQMPQEAQKIQSDLTSHEISLEEMKKHNQGKEAAQRVLSQIDVAQKKLQDVSMKFRLFQKPANFEQRLQESKMILDEVKMHLPALETKSVEQEVVQSQLNHCVNLYKSLSEVKSEVEMVIKTGRQIVQKKQTENPKELDERVTALKLHYNELGAKVTERKQQLEKCLKLSRKMRKEMNVLTEWLAATDMELTKRSAVEGMPSNLDSEVAWGKATQKEIEKQKVHLKSITEVGEALKTVLGKKETLVEDKLSLLNSNWIAVTSRAEEWLNLLLEYQKHMETFDQNVDHITKWIIQADTLLDESEKKKPQQKEDVLKRLKAELNDIRPKVDSTRDQAANLMANRGDHCRKLVEPQISELNHRFAAISHRIKTGKASIPLKELEQFNSDIQKLLEPLEAEIQQGVNLKEEDFNKDMNEDNEGTVKELLQRGDNLQQRITDERKREEIKIKQQLLQTKHNALKDLRSQRRKKALEISHQWYQYKRQADDLLKCLDDIEKKLASLPEPRDERKIKEIDRELQKKKEELNAVRRQAEGLSEDGAAMAVEPTQIQLSKRWREIESKFAQFRRLNFAQIHTVREETMMVMTEDMPLEISYVPSTYLTEITHVSQALLEVEQLLNAPDLCAKDFEDLFKQEESLKNIKDSLQQSSGRIDIIHSKKTAALQSATPVERVKLQEALSQLDFQWEKVNKMYKDRQGRFDRSVEKWRRFHYDIKIFNQWLTEAEQFLRKTQIPENWEHAKYKWYLKELQDGIGQRQTVVRTLNATGEEIIQQSSKTDASILQEKLGSLNLRWQEVCKQLSDRKKRLEEQKNILSEFQRDLNEFVLWLEEADNIASIPLEPGKEQQLKEKLEQVKLLVEELPLRQGILKQLNETGGPVLVSAPISPEEQDKLENKLKQTNLQWIKVSRALPEKQGEIEAQIKDLGQLEKKLEDLEEQLNHLLLWLSPIRNQLEIYNQPNQEGPFDVKETEIAVQAKQPDVEEILSKGQHLYKEKPATQPVKRKLEDLSSEWKAVNRLLQELRAKQPDLAPGLTTIGASPTQTVTLVTQPVVTKETAISKLEMPSSLMLEVPALADFNRAWTELTDWLSLLDQVIKSQRVMVGDLEDINEMIIKQKATMQDLEQRRPQLEELITAAQNLKNKTSNQEARTIITDRIERIQNQWDEVQEHLQNRRQQLNEMLKDSTQWLEAKEEAEQVLGQARAKLESWKEGPYTVDAIQKKITETKQLAKDLRQWQTNVDVANDLALKLLRDYSADDTRKVHMITENINASWRSIHKRVSEREAALEETHRLLQQFPLDLEKFLAWLTEAETTANVLQDATRKERLLEDSKGVKELMKQWQDLQGEIEAHTDVYHNLDENSQKILRSLEGSDDAVLLQRRLDNMNFKWSELRKKSLNIRSHLEASSDQWKRLHLSLQELLVWLQLKDDELSRQAPIGGDFPAVQKQNDVHRAFKRELKTKEPVIMSTLETVRIFLTEQPLEGLEKLYQEPRELPPEERAQNVTRLLRKQAEEVNTEWEKLNLHSADWQRKIDETLERLRELQEATDELDLKLRQAEVIKGSWQPVGDLLIDSLQDHLEKVKALRGEIAPLKENVSHVNDLARQLTTLGIQLSPYNLSTLEDLNTRWKLLQVAVEDRVRQLHEAHRDFGPASQHFLSTSVQGPWERAISPNKVPYYINHETQTTCWDHPKMTELYQSLADLNNVRFSAYRTAMKLRRLQKALCLDLLSLSAACDALDQHNLKQNDQPMDILQIINCLTTIYDRLEQEHNNLVNVPLCVDMCLNWLLNVYDTGRTGRIRVLSFKTGIISLCKAHLEDKYRYLFKQVASSTGFCDQRRLGLLLHDSIQIPRQLGEVASFGGSNIEPSVRSCFQFANNKPEIEAALFLDWMRLEPQSMVWLPVLHRVAAAETAKHQAKCNICKECPIIGFRYRSLKHFNYDICQSCFFSGRVAKGHKMHYPMVEYCTPTTSGEDVRDFAKVLKNKFRTKRYFAKHPRMGYLPVQTVLEGDNMETPVTLINFWPVDSAPASSPQLSHDDTHSRIEHYASRLAEMENSNGSYLNDSISPNESIDDEHLLIQHYCQSLNQDSPLSQPRSPAQILISLESEERGELERILADLEEENRNLQAEYDRLKQQHEHKGLSPLPSPPEMMPTSPQSPRDAELIAEAKLLRQHKGRLEARMQILEDHNKQLESQLHRLRQLLEQPQAEAKVNGTTVSSPSTSLQRSDSSQPMLLRVVGSQTSDSMGEEDLLSPPQDTSTGLEEVMEQLNNSFPSSRGRNTPGKPMREDTM

SEQ ID NO: 5 - protein, 3092 aa, Homo sapiens
MLWWEEVEDCYEREDVQKKTFTKWVNAQFSKFGKQHIENLFSDLQDGRRLLDLLEGLTGQKLPKEKGSTRVHALNNVNKALRVLQNNNVDLVNIGSTDIVDGNHKLTLGLIWNIILHWQVKNVMKNIMAGLQQTNSEKILLSWVRQSTRNYPQVNVINFTTSWSDGLALNALIHSHRPDLFDWNSVVCQQSATQRLEHAFNIARYQLGIEKLLDPEDVDTTYPDKKSILMYITSLFQVLPQQVSIEAIQEVEMLPRPPKVTKEEHFQLHHQMHYSQQITVSLAQGYERTSSPKPRFKSYAYTQAAYVTTSDPTRSPFPSQHLEAPEDKSFGSSLMESEVNLDRYQTALEEVLSWLLSAEDTLQAQGEISNDVEVVKDQFHTHEGYMMDLTAHQGRVGNILQLGSKLIGTGKLSEDEETEVQEQMNLLNSRWECLRVASMEKQSNLHRVLMDLQNQKLKELNDWLTKTEERTRKMEEEPLGPDLEDLKRQVQQHKVLQEDLEQEQVRVNSLTHMVVVVDESSGDHATAALEEQLKVLGDRWANICRWTEDRWVLLQDILLKWQRLTEEQCLFSAWLSEKEDAVNKIHTTGFKDQNEMLSSLQKLAVLKADLEKKKQSMGKLYSLKQDLLSTLKNKSVTQKTEAWLDNFARCWDNLVQKLEKSTAQISQAVTTTQPSLTQTTVMETVTTVTTREQILVKHAQEELPPPPPQKKRQITVDSEIRKRLDVDITELHSWITRSEAVLQSPEFAIFRKEGNFSDLKEKVNAIEREKAEKFRKLQDASRSAQALVEQMVNEGVNADSIKQASEQLNSRWIEFCQLLSERLNWLEYQNNIIAFYNQLQQLEQMTTTAENWLKIQPTTPSEPTAIKSQLKICKDEVNRLSDLQPQIERLKIQSIALKEKGQGPMFLDADFVAFTNHFKQVFSDVQAREKELQTIFDTLPPMRYQETMSAIRTWVQQSETKLSIPQLSVTDYEIMEQRLGELQALQSSLQEQQSGLYYLSTTVKEMSKKAPSEISRKYQSEFEEIEGRWKKLSSQLVEHCQKLEEQMNKLRKIQNHIQTLKKWMAEVDVFLKEEWPALGDSEILKKQLKQCRLLVSDIQTIQPSLNSVNEGGQKIKNEAEPEFASRLETELKELNTQWDHMCQQVYARKEALKGGLEKTVSLQKDLSEMHEWMTQAEEEYLERDFEYKTPDELQKAVEEMKRAKEEAQQKEAKVKLLTESVNSVIAQAPPVAQEALKKELETLTTNYQWLCTRLNGKCKTLEEVWACWHELLSYLEKANKWLNEVEFKLKTTENIPGGAEEISEVLDSLENLMRHSEDNPNQIRILAQTLTDGGVMDELINEELETFNSRWRELHEEAVRRQKLLEQSIQSAQETEKSLHLIQESLTFIDKQLAAYIADKVDAAQMPQEAQKIQSDLTSHEISLEEMKKHNQGKEAAQRVLSQIDVAQKKLQDVSMKFRLFQKPANFEQRLQESKMILDEVKMHLPALETKSVEQEVVQSQLNHCVNLYKSLSEVKSEVEMVIKTGRQIVQKKQTENPKELDERVTALKLHYNELGAKVTERKQQLEKCLKLSRKMRKEMNVLTEWLAATDMELTKRSAVEGMPSNLDSEVAWGKATQKEIEKQKVHLKSITEVGEALKTVLGKKETLVEDKLSLLNSNWIAVTSRAEEWLNLLLEYQKHMETFDQNVDHITKWIIQADTLLDESEKKKPQQKEDVLKRLKAELNDIRPKVDSTRDQAANLMANRGDHCRKLVEPQISELNHRFAAISHRIKTGKASIPLKELEQFNSDIQKLLEPLEAEIQQGVNLKEEDFNKDMNEDNEGTVKELLQRGDNLQQRITDERKREEIKIKQQLLQTKHNALKDLRSQRRKKALEISHQWYQYKRQADDLLKCLDDIEKKLASLPEPRDERKIKEIDRELQKKKEELNAVRRQAEGLSEDGAAMAVEPTQIQLSKRWREIESKFAQFRRLNFAQIHTVREETMMVMTEDMPLEISYVPSTYLTEITHVSQALLEVEQLLNAPDLCAKDFEDLFKQEESLKNIKDSLQQSSGRIDIIHSKKTAALQSATPVERVKLQEALSQLDFQWEKVNKMYKDRQGRFDRSVEKWRRFHYDIKIFNQWLTEAEQFLRKTQIPENWEHAKYKWYLKDLQGEIEAHTDVYHNLDENSQKILRSLEGSDDAVLLQRRLDNMNFKWSELRKKSLNIRSHLEASSDQWKRLHLSLQELLVWLQLKDDELSRQAPIGGDFPAVQKQNDVHRAFKRELKTKEPVIMSTLETVRIFLTEQPLEGLEKLYQEPRELPPEERAQNVTRLLRKQAEEVNTEWEKLNLHSADWQRKIDETLERLRELQEATDELDLKLRQAEVIKGSWQPVGDLLIDSLQDHLEKVKALRGEIAPLKENVSHVNDLARQLTTLGIQLSPYNLSTLEDLNTRWKLLQVAVEDRVRQLHEAHRDFGPASQHFLSTSVQGPWERAISPNKVPYYINHETQTTCWDHPKMTELYQSLADLNNVRFSAYRTAMKLRRLQKALCLDLLSLSAACDALDQHNLKQNDQPMDILQIINCLTTIYDRLEQEHNNLVNVPLCVDMCLNWLLNVYDTGRTGRIRVLSFKTGIISLCKAHLEDKYRYLFKQVASSTGFCDQRRLGLLLHDSIQIPRQLGEVASFGGSNIEPSVRSCFQFANNKPEIEAALFLDWMRLEPQSMVWLPVLHRVAAAETAKHQAKCNICKECPIIGFRYRSLKHFNYDICQSCFFSGRVAKGHKMHYPMVEYCTPTTSGEDVRDFAKVLKNKFRTKRYFAKHPRMGYLPVQTVLEGDNMETPVTLINFWPVDSAPASSPQLSHDDTHSRIEHYASRLAEMENSNGSYLNDSISPNESIDDEHLLIQHYCQSLNQDSPLSQPRSPAQILISLESEERGELERILADLEEENRNLQAEYDRLKQQHEHKGLSPLPSPPEMMPTSPQSPRDAELIAEAKLLRQHKGRLEARMQILEDHNKQLESQLHRLRQLLEQPQAEAKVNGTTVSSPSTSLQRSDSSQPMLLRVVGSQTSDSMGEEDLLSPPQDTSTGLEEVMEQLNNSFPSSRGRNTPGKPMREDTM

SEQ ID NO: 6 - DNA, 22 bp, Homo sapiens
aaggattatgtattacctcccg

SEQ ID NO: 7 - DNA, 22 bp, Homo sapiens
ttcctaatacataatggagggc

SEQ ID NO: 8 - DNA, 22 bp, Homo sapiens
taagattgggtatgagggatag

SEQ ID NO: 9 - DNA, 22 bp, Homo sapiens
attctaacccatactccctatc

SEQ ID NO: 10 - DNA, 22 bp, Homo sapiens
ctacatggtgtatctgactaag

SEQ ID NO: 11 - DNA, 22 bp, Homo sapiens
gatgtaccacatagactgattc

SEQ ID NO: 12 - DNA, 22 bp, Homo sapiens
ctggccgaagtataggaatatg

SEQ ID NO: 13 - DNA, 22 bp, Homo sapiens
gaccggcttcatatccttatac

SEQ ID NO: 14 - DNA, 9 bp, Homo sapiens
aaggattat

SEQ ID NO: 15 - DNA, 9 bp, Homo sapiens
ttcctaata

SEQ ID NO: 16 - DNA, 9 bp, Homo sapiens
taagattgg

SEQ ID NO: 17 - DNA, 9 bp, Homo sapiens
attctaacc

SEQ ID NO: 18 - DNA, 9 bp, Homo sapiens
ctacatggt

SEQ ID NO: 19 - DNA, 9 bp, Homo sapiens
gatgtacca

SEQ ID NO: 20 - DNA, 9 bp, Homo sapiens
ctggccgaa

SEQ ID NO: 21 - DNA, 9 bp, Homo sapiens
gaccggctt

SEQ ID NO: 22 - DNA, 9 bp, Homo sapiens
tacctcccg

SEQ ID NO: 23 - DNA, 9 bp, Homo sapiens
atggagggc

SEQ ID NO: 24 - DNA, 9 bp, Homo sapiens
gagggatag

SEQ ID NO: 25 - DNA, 9 bp, Homo sapiens
ctccctatc

SEQ ID NO: 26 - DNA, 9 bp, Homo sapiens
ctgactaag

SEQ ID NO: 27 - DNA, 9 bp, Homo sapiens
gactgattc

SEQ ID NO: 28 - DNA, 9 bp, Homo sapiens
aggaatatg

SEQ ID NO: 29 - DNA, 9 bp, Homo sapiens
tccttatac

SEQ ID NO: 30 - DNA, 22 bp, Artificial Sequence
  Synthesized
aaggattatgtatgagggatag

SEQ ID NO: 31 - DNA, 22 bp, Artificial Sequence
  Synthesized
ttcctaatacatactccctatc

SEQ ID NO: 32 - DNA, 22 bp, Artificial Sequence
  Synthesized
aaggattatgtatctgactaag

SEQ ID NO: 33 - DNA, 22 bp, Artificial Sequence
  Synthesized
ttcctaatacatagactgattc

SEQ ID NO: 34 - DNA, 22 bp, Artificial Sequence
  Synthesized
aaggattatgtataggaatatg

SEQ ID NO: 35 - DNA, 22 bp, Artificial Sequence
  Synthesized
ttcctaatacatatccttatac

SEQ ID NO: 36 - protein, 354 aa, Artificial Sequence
  Synthesized
MNTKYNKEFLLYLAGFVDSDGSIYATIRPVQSTKFKHTLRLWFAVTQKTQRRWFLDKLVDEIGVGYVYDNGSVSWYYLSEIKPLHNFLTQLQPFLKLKQKQANLVLKIIEQLPSAKESPDKFLEVCTWVDQIAALNDSKTRKTTSETVRAVLDSLPGSVGGLSPSQASSAASSASSSPGSGISEALRAGAGSGTGYNKEFLLYLAGFVDGDGSICACIVPRQDRKFKHQLRLFFEVGQKTKRRWFLDKLVDEIGVGYVEDTGRASRYRLSQIKPLHNFLTQLQPFLKLKQKQANLVLKIIEQLPSAKESPDKFLEVCTWVDQIAALNDSRTRKTTSETVRAVLDSLSEKKKSSP

SEQ ID NO: 37 - protein, 354 aa, Artificial Sequence
  Synthesized
MNTKYNKEFLLYLAGFVDSDGSIFAVIEPVQSAKFKHRLKLSFVVTQKTQRRWFLDKLVDEIGVGYVYDQGSVSFYRLSEIKPLHNFLTQLQPFLKLKQKQANLVLKIIEQLPSAKESPDKFLEVCTWVDQIAALNDSKTRKTTSETVRAVLDSLPGSVGGLSPSQASSAASSASSSPGSGISEALRAGAGSGTGYNKEFLLYLAGFVDGDGSICACIVPRQDRKFKHQLRLFFEVGQTTRRRWFLDKLVDEIGVGYVFDKGSASMYRLSEIKPLHNFLTQLQPFLKLKQKQANLVLKIIEQLPSAKESPDKFLEVCTWVDQIAALNDSRTRKTTSETVRAVLDSLSEKKKSSP

SEQ ID NO: 38 - protein, 354 aa, Artificial Sequence
  Synthesized
MNTKYNKEFLLYLAGFVDSDGSIYASIMPIQTAKFKHRLKLQFAVAQKTQRRWFLDKLVDEIGVGYVYDFGSVSYYRLSQIKPLHNFLTQLQPFLKLKQKQANLVLKIIEQLPSAKESPDKFLEVCTWVDQIAALNDSKTRKTTSETVRAVLDSLPGSVGGLSPSQASSAASSASSSPGSGISEALRAGAGSGTGYNKEFLLYLAGFVDGDGSICACIVPRQDRKFKHQLRLFFEVGQKTQRRWFLDKLVDEIGVGYVRDLGSASTYRLSEIKPLHNFLTQLQPFLKLKQKQANLVLKIIEQLPSAKESPDKFLEVCTWVDQIAALNDSRTRKTTSETVRAVLDSLSEKKKSSP

SEQ ID NO: 39 - protein, 354 aa, Artificial Sequence
  Synthesized
MNTKYNKEFLLYLAGFVDSDGSIIAFIMPSQTAKFKHRLKLQFAVAQKTQRRWFLDKLVDEIGVGYVYDFGSVSYYRLSQIKPLHNFLTQLQPFLKLKQKQANLVLKIIEQLPSAKESPDKFLEVCTWVDQIAALNDSKTRKTTSETVRAVLDSLPGSVGGLSPSQASSAASSASSSPGSGISEALRAGAGSGTGYNKEFLLYLAGFVDGDGSICACIVPRQDRKFKHQLRLFFEIGQKTQRRWFLDKLVDEIGVGYVRDLGSASTYRLSQIKPLHNFLTQLQPFLKLKQKQANLVLKIIEQLPSAKESPDKFLEVCTWVDQIAALNDSKTRKTTSETVRAVLDSLSEKKKSSP

SEQ ID NO: 40 - protein, 354 aa, Artificial Sequence
  Synthesized
MNTKYNKEFLLYLAGFVDSDGSIMAFIMPTQTAKFKHRLKLQFAVAQKTQRRWFLDKLVDEIGVGYVYDFGSVSYYRLSEIKPLHNFLTQLQPFLKLKQKQANLVLKIIEQLPSAKESPDKFLEVCTWVDQIAALNDSKTRKTTSETVRAVLDSLPGSVGGLSPSQASSAASSASSSPGSGISEALRAGAGSGTGYNKEFLLYLAGFVDGDGSICACIVPRQDRKFKHQLRLFFEVGQKTQRRWFLDKLVDEIGVGYVRDLGSASTYRLSQIKPLHNFLTQLQPFLKLKQKQANLVLKIIEQLPSAKESPDKFLEVCTWVDQIAALNDSRTRKTTSETVRAVLDSLSEKKKSSP

SEQ ID NO: 41 - protein, 354 aa, Artificial Sequence
  Synthesized
MNTKYNKEFLLYLAGFVDSDGSIMAFILPEQHMKFKHRLRLQFAVAQKTQRRWFLDKLVDEIGVGYVYDFGSVSYYRLSEIKPLHNFLTQLQPFLKLKQKQANLVLKIIEQLPSAKESPDKFLEVCTWVDQIAALNDSKTRKTTSETVRAVLDSLPGSVGGLSPSQASSAASSASSSPGSGISEALRAGAGSGTGYNKEFLLYLAGFVDGDGSICACIVPRQDRKFKHQLRLFFEVGQKTQRRWFLDKLVDEIGVGYVRDLGSASTYRLSEIKPLHNFLTQLQPFLKLKQKQANLVLKIIEQLPSAKESPDKFLEVCTWVDQIAALNDSRTRKTTSETVRAVLDSLSEKKKSSP

SEQ ID NO: 42 - protein, 354 aa, Artificial Sequence
  Synthesized
MNTKYNKEFLLYLAGFVDSDGSIMAFILPEQHLKFKHRLRLQFAVAQKTQRRWFLDKLVDEIGVGYVYDFGSVSYYRLSEIKPLHNFLTQLQPFLKLKQKQANLVLKIIEQLPSAKESPDKFLEVCTWVDQIAALNDSKTRKTTSETVRAVLDSLPGSVGGLSPSQASSAASSASSSPGSGISEALRAGAGSGTGYNKEFLLYLAGFVDGDGSICACIVPRQDRKFKHQLRLFFEVGQKTQRRWFLDKLVDEIGVGYVRDLGSASTYRLSEIKPLHNFLTQLQPFLKLKQKQANLVLKIIEQLPSAKESPDKFLEVCTWVDQIAALNDSRTRKTTSETVRAVLDSLSEKKKSSP

SEQ ID NO: 43 - protein, 354 aa, Artificial Sequence
  Synthesized
MNTKYNKEFLLYLAGFVDSDGSIMAFILPEQGLKFKHRLRLQFAVAQKTQRRWFLDKLVDEIGVGYVYDFGSVSYYRLSQIKPLHNFLTQLQPFLKLKQKQANLVLKIIEQLPSAKESPDKFLEVCTWVDQIAALNDSKTRKTTSETVRAVLDSLPGSVGGLSPSQASSAASSASSSPGSGISEALRAGAGSGTGYNKEFLLYLAGFVDGDGSICACIVPRQDRKFKHQLRLFFEVGQKTQRRWFLDKLVDEIGVGYVRDLGSASTYRLSQIKPLHNFLTQLQPFLKLKQKQANLVLKIIEQLPSAKESPDKFLEVCTWVDQIAALNDSRTRKTTSETVRAVLDSLSEKKKSSP

SEQ ID NO: 44 - protein, 354 aa, Artificial Sequence
  Synthesized
MNTKYNKEFLLYLAGFVDSDGSIMAFIMPDQAPKFKHRLRLQFAVAQKTQRRWFLDKLVDEIGVGYVYDFGSVSYYRLSEIKPLHNFLTQLQPFLKLKQKQANLVLKIIEQLPSAKESPDKFLEVCTWVDQIAALNDSKTRKTTSETVRAVLDSLPGSVGGLSPSQASSAASSASSSPGSGISEALRAGAGSGTGYNKEFLLYLAGFVDGDGSICACIVPRQDRKFKHQLRLFFEVGQKTQRRWFLDKLVDEIGVGYVRDLGSASTYRLSQIKPLHNFLTQLQPFLKLKQKQANLVLKIIEQLPSAKESPDKFLEVCTWVDQIAALNDSRTRKTTSETVRAVLDSLSEKKKSSP

SEQ ID NO: 45 - protein, 354 aa, Artificial Sequence
  Synthesized
MNTKYNKEFLLYLAGFVDADGSIYACIKPHQQLKFKHQLLLYFEVYQKTQRRWFLDKLVDEIGVGYVADRGSVSEYRLSQIKPLHNFLTQLQPFLKLKQKQANLVLKIIEQLPSAKESPDKFLEVCTWVDQIAALNDSKTRKTTSETVRAVLDSLPGSVGGLSPSQASSAASSASSSPGSGISEALRAGAGSGTGYNKEFLLYLAGFVDGDGSIFASIMPTQWTKFKHSLLLRFRVTQSTRRRWFLDKLMDEIGVGYVSDQGRASYYTLSEIKPLHNFLTQLQPFLKLKQKQANLVLKIIEQLPSAKESPDKFLEVCTWVDQIAALNDSRTRKTTSETVRAVLDSLSEKKKSSP

SEQ ID NO: 46 - protein, 354 aa, Artificial Sequence
  Synthesized
MNTKYNKEFLLYLAGFVDADGSIYACIKPHQQLKFKHQLLLYFEVYQKTQRRWFLDKLVDEIGVGYVIDSGSVSTYRLSQIKPLHNFLTQLQPFLKLKQKQANLVLKIIEQLPSAKESPDKFLEVCTWVDQIAALNDSKTRKTTSETVRAVLDSLPGSVGGLSPSQASSAASSASSSPGSGISEALRAGAGSGTGYNKEFLLYLAGFVDGDGSIFASIIPSQLVKFKHTLLLRFRVTQATRRRWFLDKLVDEIGVGYVTDNGRASYYTLSEIKPLHNFLTQLQPFLKLKQKQANLVLKIIEQLPSAKESPDKFLEVCTWVDQIAALNDSRTRKTTSETVRAVLDSLSEKKKSSP

SEQ ID NO: 47 - protein, 354 aa, Artificial Sequence
  Synthesized
MNTKYNKEFLLYLAGFVDADGSIYACIKPHQQLKFKHQLLLYFEVYQKTQRRWFLDKLVDEIGVGYVADRGSVSEYRLSQIKPLHNFLTQLQPFLKLKQKQANLVLKIIEQLPSAKESPDKFLEVCTWVDQIAALNDSKTRKTTSETVRAVLDSLPGSVGGLSPSQASSAASSASSSPGSGISEALRAGAGSGTGYNKEFLLYLAGFVDGDGSIFASIIPSQLVKFKHTLLLRFRVCQATKRRWFLDKLVDEIGVGYVSDQGSASYYTLSEIKPLHNFLTQLQPFLKLKQKQANLVLKIIEQLPSAKESPDKFLEVCTWVDQIAALNDSRTRKTTSETVRAVLDSLSEKKKSSP

SEQ ID NO: 48 - protein, 354 aa, Artificial Sequence
  Synthesized
MNTKYNKEFLLYLAGFVDSDGSIYACIKPHQQLKFKHQLLLYFEVYQKTQRRWFLDKLVDEIGVGYVADRGSVSEYRLSQIKPLHNFLTQLQPFLKLKQKQANLVLKIIEQLPSAKESPDKFLEVCTWVDQIAALNDSKTRKTTSETVRAVLDSLPGSVGGLSPSQASSAASSASSSPGSGISEALRAGAGSGTGYNKEFLLYLAGFVDGDGSIFASIIPSQEVKFKHTLLLRFRVCQATKRRWFLDKLVDEIGVGYVSDQGSASYYTLSEIKPLHNFLTQLQPFLKLKQKQANLVLKIIEQLPSAKESPDKFLEVCTWVDQIAALNDSRTRKTTSETVRAVLDSLSEKKKSSP

SEQ ID NO: 49 - protein, 354 aa, Artificial Sequence
  Synthesized
MNTKYNKEFLLYLAGFVDADGSIYACIKPHQQLKFKHQLLLYFEVYQKTQRRWFLDKLVDEIGVGYVADRGSVSEYRLSQIKPLHNFLTQLQPFLKLKQKQANLVLKIIEQLPSAKESPDKFLEVCTWVDQIAALNDSKTRKTTSETVRAVLDSLPGSVGGLSPSQASSAASSASSSPGSGISEALRAGAGSGTGYNKEFLLYLAGFVDGDGSIFASIIPSQEVKFKHTLLLRFRVCQATKRRWFLDKLVDEIGVGYVSDQGSASYYTLSEIKPLHNFLTQLQPFLKLKQKQANLVLKIIEQLPSAKESPDKFLEVCTWVDQIAALNDSRTRKTTSETVRAVLDSLSEKKKSSP

SEQ ID NO: 50 - protein, 354 aa, Artificial Sequence
  Synthesized
MNTKYNKEFLLYLAGFVDADGSIYACIKPHQQLKFKHQLLLYFEVYQKTQRRWFLDKLVDEIGVGYVADRGSVSEYRLSQIKPLHNFLTQLQPFLKLKQKQANLVLKIIEQLPSAKESPDKFLEVCTWVDQIAALNDSKTRKTTSETVRAVLDSLPGSVGGLSPSQASSAASSASSSPGSGISEALRAGAGSGTGYNKEFLLYLAGFVDGDGSIFASIIPSQEVKFKHTLLLRFRVTQATKRRWFLDKLVDEIGVGYVSDVGSASYYTLSEIKPLHNFLTQLQPFLKLKQKQANLVLKIIEQLPSAKESPDKFLEVCTWVDQIAALNDSRTRKTTSETVRAVLDSLSEKKKSSP

SEQ ID NO: 51 - protein, 354 aa, Artificial Sequence
  Synthesized
MNTKYNKEFLLYLAGFVDSDGSIYACIKPHQQLKFKHQLLLYFEVYQKTQRRWFLDKLVDEIGVGYVADRGSVSEYRLSQIKPLHNFLTQLQPFLKLKQKQANLVLKIIEQLPSAKESPDKFLEVCTWVDQIAALNDSKTRKTTSETVRAVLDSLPGSVGGLSPSQASSAASSASSSPGSGISEALRAGAGSGTGYNKEFLLYLAGFVDGDGSIFASIIPSQEVKFKHTLLLRFRVCQATKRRWFLDKLVDEIGVGYVSDRGSASYYTLSEIKPLHNFLTQLQPFLKLKQKQANLVLKIIEQLPSAKESPDKFLEVCTWVDQIAALNDSRTRKTTSETVRAVLDSLSEKKKSSP

SEQ ID NO: 52 - protein, 354 aa, Artificial Sequence
  Synthesized
MNTKYNKEFLLYLAGFVDADGSIYACIKPHQELKFKHQLLLYFEVYQKTQRRWFLDKLVDEIGVGYVADRGSVSEYRLSEIKPLHNFLTQLQPFLKLKQKQANLVLKIIEQLPSAKESPDKFLEVCTWVDQIAALNDSKTRKTTSETVRAVLDSLPGSVGGLSPSQASSAASSASSSPGSGISEALRAGAGSGTGYNKEFLLYLAGFVDGDGSIFASIIPSQEVKFKHTLLLRFRVCQATKRRWFLDKLVDEIGVGYVSDQGSASYYTLSQIKPLHNFLTQLQPFLKLKQKQANLVLKIIEQLPSAKESPDKFLEVCTWVDQIAALNDSRTRKTTSETVRAVLDSLSEKKKSSP

SEQ ID NO: 53 - protein, 354 aa, Artificial Sequence
  Synthesized
MNTKYNKEFLLYLAGFVDSDGSIVATIRPGQELKFKHGLRLRFYVCQKTQRRWFLDKLVDEIGVGYVTDSGSVSRYELSQIKPLHNFLTQLQPFLKLKQKQANLVLKIIEQLPSAKESPDKFLEVCTWVDQIAALNDSKTRKTTSETVRAVLDSLPGSVGGLSPSQASSAASSASSSPGSGISEALRAGAGSGTGYNKEFLLYLAGFVDGDGSIFACIRPSQRAKFKHVLQLCFRVHQLTKRRWFLDKLVDEIGVGYVYDCGSASFYHLSQIKPLHNFLTQLQPFLKLKQKQANLVLKIIEQLPSAKESPDKFLEVCTWVDQIAALNDSKTRKTTSETVRAVLDSLSEKKKSSP

SEQ ID NO: 54 - protein, 354 aa, Artificial Sequence
  Synthesized
MNTKYNKEFLLYLAGFVDADGSIVATIRPGQELKFKHGLRLRFYVCQKTQRRWFLDKLVDEIGAGYVTDSGSVSRYELSQIKPLHNFLTQLQPFLKLKQKQANLVLKIIEQLPSAKESPDKFLEVCTWVDQIAALNDSKTRKTTSETVRAVLDSLPGSVGGLSPSQASSAASSASSSPGSGISEALRAGAGSGTGYNKEFLLYLAGFVDGDGSIFACIRPSQRAKFKHVLQLCFRVHQKTKRRWFLDKLVDEIGVGYVYDHGSASCYHLSEIKPLHNFLTQLQPFLKLKQKQANLVLKIIEQLPSAKESPDKFLEVCTWVDQIAALNDSHTRKTTSETVRAVLDSLSEKKKSSP

SEQ ID NO: 55 - protein, 354 aa, Artificial Sequence
  Synthesized
MNTKYNKEFLLYLAGFVDADGSIVATIRPGQELKFKHGLRLRFYVCQKTQRRWFLDKLVDEIGVGYVTDSGSVSRYELSQIKPLHNFLTQLQPFLKLKQKQANLVLKIIEQLPSAKESPDKFLEVCTWVDQIAALNDSKTRKTTSETVRAVLDSLPGSVGGLSPSQASSAASSASSSPGSGISEALRAGAGSGTGYNKEFLLYLAGFVDGDGSIFACIRPSQRAKFKHVLQLCFRVHQSTRRRWFLDKLVDEIGAGYVYDHGSASLYSLSQIKPLHNFLTQLQPFLKLKQKQANLVLKIIEQLPSAKESPDKFLEVCTWVDQIAALNDSHTRKTTSETVRAVLDSLSEKKKSSP

SEQ ID NO: 56 - protein, 354 aa, Artificial Sequence
  Synthesized
MNTKYNKEFLLYLAGFVDSDGSIVASIAPAQDCKFKHRLRLRFFVSQKTQRRWFLDKLVDEIGVGYVSDSGSVSSYVLSEIKPLHNFLTQLQPFLKLKQKQANLVLKIIEQLPSAKESPDKFLEVCTWVDQIAALNDSKTRKTTSETVRAVLDSLPGSVGGLSPSQASSAASSASSSPGSGISEALRAGAGSGTGYNKEFLLYLAGFVDGDGSIFACIRPSQRAKFKHVLQLCFRVFQKTQRRWFLDKLVDEIGVGYVYDHGRASIYQLSQIKPLHNFLTQLQPFLKLKQKQANLVLKIIEQLPSAKESPDKFLEVCTWVDQIAALNDSHTRKTTSETVRAVLDSLSEKKKSSP

SEQ ID NO: 57 - protein, 354 aa, Artificial Sequence
  Synthesized
MNTKYNKEFLLYLAGFVDSDGSIVARIEPAQDCKFKHRLRLQFFVSQKTQRRWFLDKLVDEIGVGYVRDSGSVSSYDLSQIKPLHNFLTQLQPFLKLKQKQANLVLKIIEQLPSAKESPDKFLEVCTWVDQIAALNDSKTRKTTSETVRAVLDSLPGSVGGLSPSQASSAASSASSSPGSGISEALRAGAGSGTGYNKEFLLYLAGFVDGDGSIFACIRPSQRAKFKHVLQLHFRVFQKTQRRWFLDKLVDEIGVGYVYDHGRASIYQLSQIKPLHNFLTQLQPFLKLKQKQANLVLKIIEQLPSAKESPDKFLEVCTWVDQIAALNDSHTRKTTSETVRAVLDSLSEKKKSSP

SEQ ID NO: 58 - protein, 354 aa, Artificial Sequence
  Synthesized
MNTKYNKEFLLYLAGFVDSDGSIVARIEPAQDCKFKHRLRLQFFVSQKTQRRWFLDKLVDEIGVGYVRDSGSVSSYLLSQIKPLHNFLTQLQPFLKLKQKQANLVLKIIEQLPSAKESPDKFLEVCTWVDQIAALNDSKTRKTTSETVRAVLDSLPGSVGGLSPSQASSAASSASSSPGSGISEALRAGAGSGTGYNKEFLLYLAGFVDGDGSIFACIRPSQRAKFKHVLQLCFRVFQKTQRRWFLDKLVDEIGVGYVYDHGRASIYQLSQIKPLHNFLTQLQPFLKLKQKQANLVLKIIEQLPSAKESPDKFLEVCTWVDQIAALNDSHTRKTTSETVRAVLDSLSEKKKSSP

SEQ ID NO: 59 - protein, 354 aa, Artificial Sequence
  Synthesized
MNTKYNKEFLLYLAGFVDADGSIVARIEPAQDCKFKHRLRLQFFVSQKTQRRWFLDKLVDEIGVGYVRDSGSVSSYNLSEIKPLHNFLTQLQPFLKLKQKQANLVLKIIEQLPSAKESPDKFLEVCTWVDQIAALNDSKTRKTTSETVRAVLDSLPGSVGGLSPSQASSAASSASSSPGSGISEALRAGAGSGTGYNKEFLLYLAGFVDGDGSIFACIRPSQRAKFKHVLQLCFRVFQKTQRRWFLDKLVDEIGVGYVYDHGRASIYQLSQIKPLHNFLTQLQPFLKLKQKQANLVLKIIEQLPSAKESPDKFLEVCTWVDQIAALNDSHTRKTTSETVRAVLDSLSEKKKSSP

SEQ ID NO: 60 - DNA, 1065 bp, Artificial Sequence
  Synthesized
atgaatacaaaatataataaagagttcttactctacttagcagggtttgtagactctgacggttccatctatgccacgatccggcctgttcaaagtactaagttcaagcacactctgcggctctggttcgcggtcacgcagaagacacagcgccgttggttcctcgacaagctggtggacgagatcggtgtgggttacgtgtatgacaatggcagcgtctcctggtactatctgtccgagatcaagcctttgcataattttttaacacaactacaaccttttctaaaactaaaacaaaaacaagcaaatttagttttaaaaattattgaacaacttccgtcagcaaaagaatccccggacaaattcttagaagtttgtacatgggtggatcaaattgcagctctgaatgattcgaagacgcgtaaaacaacttctgaaaccgttcgtgctgtgctagacagtttaccaggatccgtgggaggtctatcgccatctcaggcatccagcgccgcatcctcggcttcctcaagcccgggttcagggatctccgaagcactcagagctggagcaggttccggcactggatacaacaaggaattcctgctctacctggcgggcttcgtcgacggggacggctccatctgtgcctgtatcgtgcctcgtcaagatcggaagttcaagcaccagctgcggctctttttcgaggtcggtcagaagacaaagcgccgttggttcctcgacaagctggtggacgagatcggtgtgggttacgtggaggacacgggcagggcgagcaggtaccggctgtcccagatcaagcctctgcacaacttcctgacccagctccagcccttcctgaagctcaagcagaagcaggccaacctcgtgctgaagatcatcgagcagctgccctccgccaaggaatccccggacaagttcctggaggtgtgcacctgggtggaccagatcgccgctctgaacgactccaggacccgcaagaccacttccgaaaccgtccgcgccgttctagacagtctctccgagaagaagaagtcgtccccctaa

SEQ ID NO: 61 - DNA, 1065 bp, Artificial Sequence
  Synthesized
atgaatacaaaatataataaagagttcttactctacttagcagggtttgtagactctgacggttccatctttgccgttatcgagcctgttcaaagtgctaagttcaagcaccggctgaagctctcgttcgttgtcactcagaagacacagcgccgttggttcctcgacaagctggtggacgagatcggtgtgggttacgtgtatgaccagggcagcgtctccttttacaggctgtccgagatcaagcctttgcataattttttaacacaactacaaccttttctaaaactaaaacaaaaacaagcaaatttagttttaaaaattattgaacaacttccgtcagcaaaagaatccccggacaaattcttagaagtttgtacatgggtggatcaaattgcagctctgaatgattcgaagacgcgtaaaacaacttctgaaaccgttcgtgctgtgctagacagtttaccaggatccgtgggaggtctatcgccatctcaggcatccagcgccgcatcctcggcttcctcaagcccgggttcagggatctccgaagcactcagagctggagcaggttccggcactggatacaacaaggaattcctgctctacctggcgggcttcgtcgacggggacggctccatctgtgcctgtatcgtgcctcgtcaagatcggaagttcaagcaccagctgcggctctttttcgaggtcgggcagacgacaaggcgccgttggttcctcgacaagctggtggacgagatcggtgtgggttacgtgtttgacaagggcagcgcgagcatgtaccggctgtccgagatcaagcctctgcacaacttcctgacccagctccagcccttcctgaagctcaagcagaagcaggccaacctcgtgctgaagatcatcgagcagctgccctccgccaaggaatccccggacaagttcctggaggtgtgcacctgggtggaccagatcgccgctctgaacgactccaggacccgcaagaccacttccgaaaccgtccgcgccgttctagacagtctctccgagaagaagaagtcgtccccctaa

SEQ ID NO: 62 - DNA, 1065 bp, Artificial Sequence
  Synthesized
atgaatacaaaatataataaagagttcttactctacttagcagggtttgtagactctgacggttccatctatgccagtatcatgcctattcaaacggctaagttcaagcaccgtctgaagctccagttcgcggtcgctcagaagacacagcgccgttggttcctcgacaagctggtggacgagatcggtgtgggttacgtgtatgactttggcagcgtctcctattacaggctgtcccagatcaagcctttgcataattttttaacacaactacaaccttttctaaaactaaaacaaaaacaagcaaatttagttttaaaaattattgaacaacttccgtcagcaaaagaatccccggacaaattcttagaagtttgtacatgggtggatcaaattgcagctctgaatgattcgaagacgcgtaaaacaacttctgaaaccgttcgtgctgtgctagacagtttaccaggatccgtgggaggtctatcgccatctcaggcatccagcgccgcatcctcggcttcctcaagcccgggttcagggatctccgaagcactcagagctggagcaggttccggcactggatacaacaaggaattcctgctctacctggcgggcttcgtcgacggggacggctccatctgtgcctgtatcgtgcctcgtcaagatcggaagttcaagcaccagctgcggctctttttcgaggtcggtcagaagacacagcgccgttggttcctcgacaagctggtggacgagatcggtgtgggttacgtgagggaccttggcagcgcgagcacttaccgtctgtccgagatcaagcctctgcacaacttcctgacccagctccagcccttcctgaagctcaagcagaagcaggccaacctcgtgctgaagatcatcgagcagctgccctccgccaaggaatccccggacaagttcctggaggtgtgcacctgggtggaccagatcgccgctctgaacgactccaggacccgcaagaccacttccgaaaccgtccgcgccgttctagacagtctctccgagaagaagaagtcgtccccctaa

SEQ ID NO: 63 - DNA, 1065 bp, Artificial Sequence
  Synthesized
atgaatacaaaatataataaagagttcttactctacttagcagggtttgtagactctgacggttccatcattgcctttatcatgcctagtcagacggctaagttcaagcaccgtctgaagctccagttcgcggtcgctcagaagacacagcgccgttggttcctcgacaagctggtggacgagatcggtgtgggttacgtgtatgactttggcagcgtctcctattacaggctgtcccagatcaagcctttgcataattttttaacacaactacaaccttttctaaaactaaaacaaaaacaagcaaatttagttttaaaaattattgaacaacttccgtcagcaaaagaatccccggacaaattcttagaagtttgtacatgggtggatcaaattgcagctctgaatgattcgaagacgcgtaaaacaacttctgaaaccgttcgtgctgtgctagacagtttaccaggatccgtgggaggtctatcgccatctcaggcatccagcgccgcatcctcggcttcctcaagcccgggttcagggatctccgaagcactcagagctggagcaggttccggcactggatacaacaaggaattcctgctctacctggcgggcttcgtcgacggggacggctccatctgtgcctgtatcgtgcctcgtcaagatcggaagttcaagcaccagctgcggctctttttcgagatcggtcagaagacacagcgccgttggttcctcgacaagctggtggacgagatcggtgtgggttacgtgagggaccttggcagcgcgagcacttaccgtctgtcccagatcaagcctctgcacaacttcctgacccagctccagcccttcctgaagctcaagcagaagcaggccaacctcgtgctgaagatcatcgagcagctgccctccgccaaggaatccccggacaagttcctggaggtgtgcacctgggtggaccagatcgccgctctgaacgactccaagacccgcaagaccacttccgaaaccgtccgcgccgttctagacagtctctccgagaagaagaagtcgtccccctaa

SEQ ID NO: 64 - DNA, 1065 bp, Artificial Sequence
  Synthesized
atgaatacaaaatataataaagagttcttactctacttagcagggtttgtagactctgacggttccatcatggcctttatcatgcctactcagacggctaagttcaagcaccgtctgaagctccagttcgcggtcgctcagaagacacagcgccgttggttcctcgacaagctggtggacgagatcggtgtgggttacgtgtatgactttggcagcgtctcctattacaggctgtccgagatcaagcctttgcataattttttaacacaactacaaccttttctaaaactaaaacaaaaacaagcaaatttagttttaaaaattattgaacaacttccgtcagcaaaagaatccccggacaaattcttagaagtttgtacatgggtggatcaaattgcagctctgaatgattcgaagacgcgtaaaacaacttctgaaaccgttcgtgctgtgctagacagtttaccaggatccgtgggaggtctatcgccatctcaggcatccagcgccgcatcctcggcttcctcaagcccgggttcagggatctccgaagcactcagagctggagcaggttccggcactggatacaacaaggaattcctgctctacctggcgggcttcgtcgacggggacggctccatctgtgcctgtatcgtgcctcgtcaagatcggaagttcaagcaccagctgcggctctttttcgaggtcggtcagaagacacagcgccgttggttcctcgacaagctggtggacgagatcggtgtgggttacgtgagggaccttggcagcgcgagcacttaccgtctgtcccagatcaagcctctgcacaacttcctgacccagctccagcccttcctgaagctcaagcagaagcaggccaacctcgtgctgaagatcatcgagcagctgccctccgccaaggaatccccggacaagttcctggaggtgtgcacctgggtggaccagatcgccgctctgaacgactccaggacccgcaagaccacttccgaaaccgtccgcgccgttctagacagtctctccgagaagaagaagtcgtccccctaa

SEQ ID NO: 65 - DNA, 1065 bp, Artificial Sequence
  Synthesized
atgaatacaaaatataataaagagttcttactctacttagcagggtttgtagactctgacggttccatcatggcctttatcttgcctgagcagcatatgaagttcaagcaccgtctgaggctccagttcgcggtcgctcagaagacacagcgccgttggttcctcgacaagctggtggacgagatcggtgtgggttacgtgtatgactttggcagcgtctcctattacaggctgtccgagatcaagcctttgcataattttttaacacaactacaaccttttctaaaactaaaacaaaaacaagcaaatttagttttaaaaattattgaacaacttccgtcagcaaaagaatccccggacaaattcttagaagtttgtacatgggtggatcaaattgcagctctgaatgattcgaagacgcgtaaaacaacttctgaaaccgttcgtgctgtgctagacagtttaccaggatccgtgggaggtctatcgccatctcaggcatccagcgccgcatcctcggcttcctcaagcccgggttcagggatctccgaagcactcagagctggagcaggttccggcactggatacaacaaggaattcctgctctacctggcgggcttcgtcgacggggacggctccatctgtgcctgtatcgtgcctcgtcaagatcggaagttcaagcaccagctgcggctctttttcgaggtcggtcagaagacacagcgccgttggttcctcgacaagctggtggacgagatcggtgtgggttacgtgagggaccttggcagcgcgagcacttaccgtctgtccgagatcaagcctctgcacaacttcctgacccagctccagcccttcctgaagctcaagcagaagcaggccaacctcgtgctgaagatcatcgagcagctgccctccgccaaggaatccccggacaagttcctggaggtgtgcacctgggtggaccagatcgccgctctgaacgactccaggacccgcaagaccacttccgaaaccgtccgcgccgttctagacagtctctccgagaagaagaagtcgtccccctaa

SEQ ID NO: 66 - DNA, 1065 bp, Artificial Sequence
  Synthesized
atgaatacaaaatataataaagagttcttactctacttagcagggtttgtagactctgacggttccatcatggcctttatcttgcctgagcagcatcttaagttcaagcaccgtctgaggctccagttcgcggtcgctcagaagacacagcgccgttggttcctcgacaagctggtggacgagatcggtgtgggttacgtgtatgactttggcagcgtctcctattacaggctgtccgagatcaagcctttgcataattttttaacacaactacaaccttttctaaaactaaaacaaaaacaagcaaatttagttttaaaaattattgaacaacttccgtcagcaaaagaatccccggacaaattcttagaagtttgtacatgggtggatcaaattgcagctctgaatgattcgaagacgcgtaaaacaacttctgaaaccgttcgtgctgtgctagacagtttaccaggatccgtgggaggtctatcgccatctcaggcatccagcgccgcatcctcggcttcctcaagcccgggttcagggatctccgaagcactcagagctggagcaggttccggcactggatacaacaaggaattcctgctctacctggcgggcttcgtcgacggggacggctccatctgtgcctgtatcgtgcctcgtcaagatcggaagttcaagcaccagctgcggctctttttcgaggtcggtcagaagacacagcgccgatggttcctcgacaagctggtggacgagatcggtgtgggttacgtgagggaccttggcagcgcgagcacttaccgtctgtccgagatcaagcctctgcacaacttcctgacccagctccagcccttcctgaagctcaagcagaagcaggccaacctcgtgctgaagatcatcgagcagctgccctccgccaaggaatccccggacaagttcctggaggtgtgcacctgggtggaccagatcgccgctctgaacgactccaggacccgcaagaccacttccgaaaccgtccgcgccgttctagacagtctctccgagaagaagaagtcgtccccctaa

SEQ ID NO: 67 - DNA, 1065 bp, Artificial Sequence
  Synthesized
atgaatacaaaatataataaagagttcttactctacttagcagggtttgtagactctgacggttccatcatggcctttatcttgcctgagcagggtctgaagttcaagcaccgtctgaggctccagttcgcggtcgctcagaagacacagcgccgttggttcctcgacaagctggtggacgagatcggtgtgggttacgtgtatgactttggcagcgtctcctattacaggctgtcccagatcaagcctttgcataattttttaacacaactacaaccttttctaaaactaaaacaaaaacaagcaaatttagttttaaaaattattgaacaacttccgtcagcaaaagaatccccggacaaattcttagaagtttgtacatgggtggatcaaattgcagctctgaatgattcgaagacgcgtaaaacaacttctgaaaccgttcgtgctgtgctagacagtttaccaggatccgtgggaggtctatcgccatctcaggcatccagcgccgcatcctcggcttcctcaagcccgggttcagggatctccgaagcactcagagctggagcaggttccggcaccggatacaacaaggaattcctgctctacctggcgggcttcgtcgacggggacggctccatctgtgcctgtatcgtgcctcgtcaagatcggaagttcaagcaccagctgcggctctttttcgaggtcggtcagaagacacagcgccgttggttcctcgacaagctggtggacgagatcggtgtgggttacgtgagggaccttggcagcgcgagcacttaccgtctgtcccagatcaagcctctgcacaacttcctgacccagctccagcccttcctgaagctcaagcagaagcaggccaacctcgtgctgaagatcatcgagcagctgccctccgccaaggaatccccggacaagttcctggaggtgtgcacctgggtggaccagatcgccgctctgaacgactccaggacccgcaagaccacttccgaaaccgtccgcgccgttctagacagtctctccgagaagaagaagtcgtccccctaa

SEQ ID NO: 68 - DNA, 1065 bp, Artificial Sequence
  Synthesized
atgaatacaaaatataataaagagttcttactctacttagcagggtttgtagactctgacggttccatcatggcctttatcatgcctgatcaggcgcctaagttcaagcaccgtctgaggctccagttcgcggtcgctcagaagacacagcgccgttggttcctcgacaagctggtggacgagatcggtgtgggttacgtgtatgactttggcagcgtctcctattacaggctgtccgagatcaagcctttgcataattttttaacacaactacaaccttttctaaaactaaaacaaaaacaagcaaatttagttttaaaaattattgaacaacttccgtcagcaaaagaatccccggacaaattcttagaagtttgtacatgggtggatcaaattgcagctctgaatgattcgaagacgcgtaaaacaacttctgaaaccgttcgtgctgtgctagacagtttaccaggatccgtgggaggtctatcgccatctcaggcatccagcgccgcatcctcggcttcctcaagcccgggttcagggatctccgaagcactcagagctggagcaggttccggcactggatacaacaaggaattcctgctctacctggcgggcttcgtcgacggggacggctccatctgtgcctgtatcgtgcctcgtcaagatcggaagttcaagcaccagctgcggctctttttcgaggtcggtcagaagacacagcgccgttggttcctcgacaagctggtggacgagatcggtgtgggttacgtgagggaccttggcagcgcgagcacttaccgtctgtcccagatcaagcctctgcacaacttcctgacccagctccagcccttcctgaagctcaagcagaagcaggccaacctcgtgctgaagatcatcgagcagctgccctccgccaaggaatccccggacaagttcctggaggtgtgcacctgggtggaccagatcgccgctctgaacgactccaggacccgcaagaccacttccgaaaccgtccgcgccgttctagacagtctctccgagaagaagaagtcgtccccctaa

SEQ ID NO: 69 - DNA, 1065 bp, Artificial Sequence
  Synthesized
atgaatacaaaatataataaagagttcttactctacttagcagggtttgtagacgctgacggttccatctatgcctgtatcaagcctcatcaacagcttaagttcaagcaccagctgttgctctatttcgaggtctatcagaagacacagcgccgttggttcctcgacaagctggtggacgagatcggtgtgggttacgtggctgaccgtggcagcgtctccgagtaccgtctgtcccagatcaagcctttgcataattttttaacacaactacaaccttttctaaaactaaaacaaaaacaagcaaatttagttttaaaaattattgaacaacttccgtcagcaaaagaatccccggacaaattcttagaagtttgtacatgggtggatcaaattgcagctctgaatgattcgaagacgcgtaaaacaacttctgaaaccgttcgtgctgtgctagacagtttaccaggatccgtgggaggtctatcgccatctcaggcatccagcgccgcatcctcggcttcctcaagcccgggttcagggatctccgaagcactcagagctggagcaggttccggcactggatacaacaaggaattcctgctctacctggcgggcttcgtcgacggggacggctccatctttgcctctatcatgccgacgcagtggacgaagttcaagcactcgctgttgctccggttccgggtcacccagtcgacaaggcgccgttggttcctcgacaagctgatggacgagattggtgtgggttacgtgtctgaccagggcagggcgagctactacaccctgtccgagatcaagcctctgcacaacttcctgacccagctccagcccttcctgaagctcaagcagaagcaggccaacctcgtgctgaagatcatcgagcagctgccctccgccaaggaatccccggacaagttcctggaggtgtgcacctgggtggaccagatcgccgctctgaacgactccaggacccgcaagaccacttccgaaaccgtccgcgccgttctagacagtctctccgagaagaagaagtcgtccccctaa

SEQ ID NO: 70 - DNA, 1065 bp, Artificial Sequence
  Synthesized
atgaatacaaaatataataaagagttcttactctacttagcagggtttgtagacgctgacggttccatctatgcctgtatcaagcctcatcaacagcttaagttcaagcaccagctgttgctctatttcgaggtctatcagaagacacagcgccgttggttcctcgacaagctggtggacgagatcggtgtgggttacgtgattgactcgggcagcgtctccacgtaccggctgtcccagatcaagcctttgcataattttttaacacaactacaaccttttctaaaactaaaacaaaaacaagcaaatttagttttaaaaattattgaacaacttccgtcagcaaaagaatccccggacaaattcttagaagtttgtacatgggtggatcaaattgcagctctgaatgattcgaagacgcgtaaaacaacttctgaaaccgttcgtgctgtgctagacagtttaccaggatccgtgggaggtctatcgccatctcaggcatctagcgccgcatcctcggcttcctcaagcccgggttcagggatctccgaagcactcagagctggagcaggttccggcactggatacaacaaggaattcctgctctacctggcgggcttcgtcgacggggacggctccatctttgcctctatcattccgtcgcagctggttaagttcaagcacactctgctgctccgtttccgggtcacccaggcgacaaggcgccgttggttcctcgacaagctggtggacgagatcggtgtgggttacgtgacggacaacggcagggcgagctactacaccctgtccgagatcaagcctctgcacaacttcctgacccagctccagcccttcctgaagctcaagcagaagcaggccaacctcgtgctgaagatcatcgagcagctgccctccgccaaggaatccccggacaagttcctggaggtgtgcacctgggtggaccagatcgccgctctgaacgactccaggacccgcaagaccacttccgaaaccgtccgcgccgttctagacagtctctccgagaagaagaagtcgtccccctaa

SEQ ID NO: 71 - DNA, 1065 bp, Artificial Sequence
  Synthesized
atgaatacaaaatataataaagagttcttactctacttagcagggtttgtagacgctgacggttccatctatgcctgtatcaagcctcatcaacagcttaagttcaagcaccagctgttgctctatttcgaggtctatcagaagacacagcgccgttggttcctcgacaagctggtggacgagatcggtgtgggttacgtggctgaccgtggcagcgtctccgagtaccgtctgtcccagatcaagcctttgcataattttttaacacaactacaaccttttctaaaactaaaacaaaaacaagcaaatttagttttaaaaattattgaacaacttccgtcagcaaaagaatccccggacaaattcttagaagtttgtacatgggtggatcaaattgcagctctgaatgattcgaagacgcgtaaaacaacttctgaaaccgttcgtgctgtgctagacagtttaccaggatccgtgggaggtctatcgccatctcaggcatccagcgccgcatcctcggcttcctcaagcccgggttcagggatctccgaagcactcagagctggagcaggttccggcactggatacaacaaggaattcctgctctacctggcgggcttcgtcgacggggacggctccatctttgcctctatcattccgtcgcagctggttaagttcaagcacactctgctgctccgtttccgggtctgccaggcgacaaagcgccgttggttcctcgacaagctggtggacgagattggtgtgggttacgtgtctgaccagggcagcgcgagctactacaccctgtccgagatcaagcctctgcacaacttcctgacccagctccagcccttcctgaagctcaagcagaagcaggccaacctcgtgctgaagatcatcgagcagctgccctccgccaaggaatccccggacaagttcctggaggtgtgcacctgggtggaccagatcgccgctctgaacgactccaggacccgcaagaccacttccgaaaccgtccgcgccgttctagacagtctctccgagaagaagaagtcgtccccctaa

SEQ ID NO: 72 - DNA, 1065 bp, Artificial Sequence
  Synthesized
atgaatacaaaatataataaagagttcttactctacttagcagggtttgtagactctgacggttccatctatgcctgtatcaagcctcatcaacagcttaagttcaagcaccagctgttgctctatttcgaggtctatcagaagacacagcgccgttggttcctcgacaagctggtggacgagatcggtgtgggttacgtggctgaccgtggcagcgtctccgagtaccgtctgtcccagatcaagcctttgcataattttttaacacaactacaaccttttctaaaactaaaacaaaaacaagcaaatttagttttaaaaattattgaacaacttccgtcagcaaaagaatccccggacaaattcttagaagtttgtacatgggtggatcaaattgcagctctgaatgattcgaagacgcgtaaaacaacttctgaaaccgttcgtgctgtgctagacagtttaccaggatccgtgggaggtctatcgccatctcaggcatccagcgccgcatcctcggcttcctcaagcccgggttcagggatctccgaagcactcagagctggagcaggttccggcactggatacaacaaggaattcctgctctacctggcgggcttcgtcgacggggacggctccatctttgcctctatcattccgtcgcaggaggttaagttcaagcacactctgctgctccgtttccgggtctgccaggcgacaaagcgccgttggttcctcgacaagctggtggacgagattggtgtgggttacgtgtctgaccagggcagcgcgagctactacaccctgtccgagatcaagcctctgcacaacttcctgacccagctccagcccttcctgaagctcaagcagaagcaggccaacctcgtgctgaagatcatcgagcagctgccctccgccaaggaatccccggacaagttcctggaggtgtgcacctgggtggaccagatcgccgctctgaacgactccaggacccgcaagaccacttccgaaaccgtccgcgccgttctagacagtctctccgagaagaagaagtcgtccccctaa

SEQ ID NO: 73 - DNA, 1065 bp, Artificial Sequence
  Synthesized
atgaatacaaaatataataaagagttcttactctacttagcagggtttgtagacgctgacggttccatctatgcctgtatcaagcctcatcaacagcttaagttcaagcaccagctgttgctctatttcgaggtctatcagaagacacagcgccgttggttcctcgacaagctggtggacgagatcggtgtgggttacgtggctgaccgtggcagcgtctccgagtaccgtctgtcccagatcaagcctttgcataattttttaacacaactacaaccttttctaaaactaaaacaaaaacaagcaaatttagttttaaaaattattgaacaacttccgtcagcaaaagaatccccggacaaattcttagaagtttgtacatgggtggatcaaattgcagctctgaatgattcgaagacgcgtaaaacaacttctgaaaccgttcgtgctgtgctagacagtttaccaggatccgtgggaggtctatcgccatctcaggcatccagcgccgcatcctcggcttcctcaagcccgggttcagggatctccgaagcactcagagctggagcaggttccggcactggatacaacaaggaattcctgctctacctggcgggcttcgtcgacggggacggctccatctttgcctctatcattccgtcgcaggaggttaagttcaagcacactctgctgctccgtttccgggtctgccaggcgacaaagcgccgttggttcctcgacaagctggtggacgagattggtgtgggttacgtgtctgaccagggcagcgcgagctactacaccctgtccgagatcaagcctctgcacaacttcctgacccagctccagcccttcctgaagctcaagcagaagcaggccaacctcgtgctgaagatcatcgagcagctgccctccgccaaggaatccccggacaagttcctggaggtgtgcacctgggtggaccagatcgccgctctgaacgactccaggacccgcaagaccacttccgaaaccgtccgcgccgttctagacagtctctccgagaagaagaagtcgtccccctaa

SEQ ID NO: 74 - DNA, 1065 bp, Artificial Sequence
  Synthesized
atgaatacaaaatataataaagagttcttactctacttagcagggtttgtagacgctgacggttccatctatgcctgtatcaagcctcatcaacagcttaagttcaagcaccagctgttgctctatttcgaggtctatcagaagacacagcgccgttggttcctcgacaagctggtggacgagatcggtgtgggttacgtggctgaccgtggcagcgtctccgagtaccgtctgtcccagatcaagcctttgcataattttttaacacaactacaaccttttctaaaactaaaacaaaaacaagcaaatttagttttaaaaattattgaacaacttccgtcagcaaaagaatccccggacaaattcttagaagtttgtacatgggtggatcaaattgcagctctgaatgattcgaagacgcgtaaaacaacttctgaaaccgttcgtgctgtgctagacagtttaccaggatccgtgggaggtctatcgccatctcaggcatccagcgccgcatcctcggcttcctcaagcccgggttcagggatctccgaagcactcagagctggagcaggttccggcactggatacaacaaggaattcctgctctacctggcgggcttcgtcgacggggacggctccatctttgcctctatcattccgtcgcaggaggttaagttcaagcacactctgctgctccgtttcagggtcactcaggcgacaaagcgccgttggttcctcgacaagctggtggacgagattggtgtgggttacgtgtctgacgttggcagcgcgagctattacaccctgtccgagatcaagcctctgcacaacttcctgacccagctccagcccttcctgaagctcaagcagaagcaggccaacctcgtgctgaagatcatcgagcagctgccctccgccaaggaatccccggacaagttcctggaggtgtgcacctgggtggaccagatcgccgctctgaacgactccaggacccgcaagaccacttccgaaaccgtccgcgccgttctagacagtctctccgagaagaagaagtcgtccccctaa

SEQ ID NO: 75 - DNA, 1065 bp, Artificial Sequence
  Synthesized
atgaatacaaaatataataaagagttcttactctacttagcagggtttgtagactctgacggttccatctatgcctgtatcaagcctcatcaacagcttaagttcaagcaccagctgttgctctatttcgaggtctatcagaagacacagcgccgttggttcctcgacaagctggtggacgagatcggtgtgggttacgtggctgaccgtggcagcgtctccgagtaccgtctgtcccagatcaagcctttgcataattttttaacacaactacaaccttttctaaaactaaaacaaaaacaagcaaatttagttttaaaaattattgaacaacttccgtcagcaaaagaatccccggacaaattcttagaagtttgtacatgggtggatcaaattgcagctctgaatgattcgaagacgcgtaaaacaacttctgaaaccgttcgtgctgtgctagacagtttaccaggatccgtgggaggtctatcgccatctcaggcatccagcgccgcatcctcggcttcctcaagcccgggttcagggatctccgaagcactcagagctggagcaggttccggcactggatacaacaaggaattcctgctctacctggcgggcttcgtcgacggggacggctccatctttgcctctatcattccgtcgcaggaggttaagttcaagcacactctgctgctccgtttccgggtctgccaggcgacaaagcgccgttggttcctcgacaagctggtggacgagattggtgtgggttacgtgtctgaccgtggcagcgcgagctattacaccctgtccgagatcaagcctctgcacaacttcctgacccagctccagcccttcctgaagctcaagcagaagcaggccaacctcgtgctgaagatcatcgagcagctgccctccgccaaggaatccccggacaagttcctggaggtgtgcacctgggtggaccagatcgccgctctgaacgactccaggacccgcaagaccacttccgaaaccgtccgcgccgttctagacagtctctccgagaagaagaagtcgtccccctaa

SEQ ID NO: 76 - DNA, 1065 bp, Artificial Sequence
  Synthesized
atgaatacaaaatataataaagagttcttactctacttagcagggtttgtagacgctgacggttccatctatgcctgtatcaagcctcatcaagagcttaagttcaagcaccagctgttgctctatttcgaggtctatcagaagacacagcgccgttggttcctcgacaagctggtggacgagatcggtgtgggttacgtggctgaccgtggcagcgtctccgagtaccgtctgtccgagatcaagcctttgcataattttttaacacaactacaaccttttctaaaactaaaacaaaaacaagcaaatttagttttaaaaattattgaacaacttccgtcagcaaaagaatccccggacaaattcttagaagtttgtacatgggtggatcaaattgcagctctgaatgattcgaagacgcgtaaaacaacttctgaaaccgttcgtgctgtgctagacagtttaccaggatccgtgggaggtctatcgccatctcaggcatccagcgccgcatcctcggcttcctcaagcccgggttcagggatctccgaagcactcagagctggagcaggttccggcactggatacaacaaggaattcctgctctacctggcgggcttcgtcgacggggacggctccatctttgcctctatcattccgtcgcaggaggttaagttcaagcacactctgctgctccgtttccgggtctgccaggcgacaaagcgccgttggttcctcgacaagctggtggacgagattggtgtgggttacgtgtctgaccagggcagcgcgagctactacaccctgtcccagatcaagcctctgcacaacttcctgacccagctccagcccttcctgaagctcaagcagaagcaggccaacctcgtgctgaagatcatcgagcagctgccctccgccaaggaatccccggacaagttcctggaggtgtgcacctgggtggaccagatcgccgctctgaacgactccaggacccgcaagaccacttccgaaaccgtccgcgccgttctagacagtctctccgagaagaagaagtcgtccccctaa

SEQ ID NO: 77 - DNA, 1065 bp, Artificial Sequence
  Synthesized
atgaatacaaaatataataaagagttcttactctacttagcagggtttgtagactctgacggttccatcgtggccactatccggccggggcaggagctgaagttcaagcacggtctgcggctcaggttctatgtctgtcagaagacacagcgccgttggttcctcgacaagctggtggacgagatcggtgtgggttacgtgacggacagtggcagcgtctcccgttacgagctgtcccagatcaagcctttgcataattttttaacacaactacaaccttttctaaaactaaaacaaaaacaagcaaatttagttttaaaaattattgaacaacttccgtcagcaaaagaatccccggacaaattcttagaagtttgtacatgggtggatcaaattgcagctctgaatgattcgaagacgcgtaagacaacttctgaaaccgttcgtgctgtgctagacagtttaccaggatccgtgggaggtctatcgccatctcaggcatccagcgccgcatcctcggcttcctcaagcccgggttcagggatctccgaagcactcagagctggagcaggttccggcactggatacaacaaggaattcctgctctacctggcgggcttcgtcgacggggacggctccatctttgcctgtatccgtccgtcgcagagggctaagttcaagcacgtgctgcagctctgtttcagggtccaccagttgacaaagcgccgttggttcctcgacaagctggtggacgagatcggtgtaggttacgtgtatgactgcggcagcgcgagcttctaccacctgtcccagatcaagcctctgcacaacttcctgacccagctccagcccttcctgaagctcaagcagaagcaggccaacctcgtgctgaagatcatcgagcagctgccctccgccaaggaatccccggacaagttcctggaggtgtgcacctgggtggaccagatcgccgctctgaacgactccaagacccgcaagaccacttccgaaaccgtccgcgccgttctagacagtctctccgagaagaagaagtcgtccccctaa

SEQ ID NO: 78 - DNA, 1065 bp, Artificial Sequence
  Synthesized
atgaatacaaaatataataaagagttcttactctacttagcagggtttgtagacgctgacggttccatcgtggccactatccggccggggcaggagctgaagttcaagcacggtctgcggctcaggttctatgtctgtcagaagacacagcgccgttggttcctcgacaagctggtggacgagatcggtgcgggttacgtgacggacagtggcagcgtctcccgttacgagctgtcccagatcaagcctttgcataattttttaacacaactacaaccttttctaaaactaaaacaaaaacaagcaaatttagttttaaaaattatcgaacaacttccgtcagcaaaagaatccccggacaaattcttagaagtttgtacatgggtggatcaaattgcagctctgaatgattcgaagacgcgtaaaacaacttctgaaaccgttcgtgctgtgctagacagtttaccaggatccgtgggaggtctatcgccatctcaggcatccagcgccgcatcctcggcttcctcaagcccgggttcagggatctccgaagcactcagagctggagcaggttccggcactggatacaacaaggaattcctgctctacctggcgggcttcgtcgacggggacggctccatctttgcctgtatccgtccgtcgcagagggctaagttcaagcacgtgctgcagctctgtttcagggtccaccagaagacaaagcgccgttggttcctcgacaagctggtggacgagatcggtgtgggttacgtgtatgaccacggcagcgcgagctgctaccacctgtccgagatcaagcctctgcacaacttcctgacccagctccagcccttcctgaagctcaagcagaagcaggccaacctcgtgctgaagatcatcgagcagctgccctccgccaaggaatccccggacaagttcctggaggtgtgcacctgggtggaccagatcgccgctctgaacgactcccacacccgcaagaccacttccgaaaccgtccgcgccgttctagacagtctctccgagaagaagaagtcgtccccctaa

SEQ ID NO: 79 - DNA, 1065 bp, Artificial Sequence
  Synthesized
atgaatacaaaatataataaagagttcttactctacttagcagggtttgtagacgctgacggttccatcgtggccactatccggccggggcaggagctgaagttcaagcacggtctgcggctcaggttctatgtctgtcagaagacacagcgccgttggttcctcgacaagctggtggacgagatcggtgtgggttacgtgacggacagtggcagcgtctcccgttacgagctgtcccagatcaagcctttgcataattttttaacacaactacaaccttttctaaaactaaaacaaaaacaagcaaatttagttttaaaaattattgaacaacttccgtcagcaaaagaatccccggacaaattcttagaagtttgtacatgggtggatcaaattgcagctctgaatgattcgaagacgcgtaaaacaacttctgaaaccgttcgtgctgtgctagacagtttaccaggatccgtgggaggtctatcgccatctcaggcatccagcgccgcatcctcggcttcctcaagcccgggttcagggatctccgaagcactcagagctggagcaggttccggcactggatacaacaaggaattcctgctctacctggcgggcttcgtcgacggggacggctccatctttgcctgtatccgtccgtcgcagagggctaagttcaagcacgtgctgcagctctgtttcagggtccaccagtcgacaaggcgccgttggttcctagacaagctggtggacgagatcggtgcgggttacgtgtatgaccacggcagcgcgagcctgtacagcctgtcccagatcaagcctctgcacaacttcctgacccagctccagcccttcctgaagctcaagcagaagcaggccaacctcgtgctgaagatcatcgagcagctgccctccgccaaggaatccccggacaagttcctggaggtgtgcacctgggtggaccagatcgccgctctgaacgactcccacacccgcaagaccacttccgaaaccgtccgcgccgttctagacagtctctccgagaagaagaagtcgtccccctaa

SEQ ID NO: 80 - DNA, 1065 bp, Artificial Sequence
  Synthesized
atgaatacaaaatataataaagagttcttactctacttagcagggtttgtagactctgacggttccatcgttgccagtatcgctccggctcaggattgtaagttcaagcacaggctgaggctccgtttctttgtctctcagaagacacagcgccgttggttcctcgacaagctggtggacgagatcggtgtgggttacgtgtctgactctggcagcgtctccagttacgttctgtccgagatcaagcctttgcataattttttaacacaactacaaccttttctaaaactaaaacaaaaacaagcaaatttagttttaaaaattattgaacaacttccgtcagcaaaagaatccccggacaaattcttagaagtttgtacatgggtggatcaaattgcagctctgaatgattcgaagacgcgtaaaacaacttctgaaaccgttcgtgctgtgctagacagtttaccaggatccgtgggaggtctatcgccatctcaggcatccagcgccgcatcctcggcttcctcaagcccgggttcagggatctccgaagcactcagagctggagcaggttccggcactggatacaacaaggaattcctgctctacctggcgggcttcgtcgacggggacggctccatctttgcctgtatccgtccgtcgcagagggctaagttcaagcacgtgctgcagctctgtttccgggtctttcagaagacacagcgccgttggttcctcgacaagctggtggacgagatcggtgtaggttacgtgtatgaccacggcagggcgagcatctaccagctgtcccagatcaagcctctgcacaacttcctgacccagctccagcccttcctgaagctcaagcagaagcaggccaacctcgtgctgaagatcatcgagcagctgccctccgccaaggaatccccggacaagttcctggaggtgtgcacctgggtggaccagatcgccgctctgaacgactcccacacccgcaagaccacttccgaaaccgtccgcgccgttctagacagtctctccgagaagaagaagtcgtccccctaa

SEQ ID NO: 81 - DNA, 1065 bp, Artificial Sequence
  Synthesized
atgaatacaaaatataataaagagttcttactctacttagcagggtttgtagactctgacggttccatcgttgccaggatcgagccggctcaggattgtaagttcaagcacaggctgaggctccagttctttgtctctcagaagacacagcgccgttggttcctcgacaagctggtggacgagatcggtgtgggttacgtgcgggactctggcagcgtctccagttacgatctgtcccagatcaagcctttgcataattttttaacacaactacaaccttttctaaaactaaaacaaaaacaagcaaatttagttttaaaaattattgaacaacttccgtcagcaaaagaatccccggacaaattcttagaagtttgtacatgggtggatcaaattgcagctctgaatgattcgaagacgcgtaaaacaacttctgaaaccgttcgtgctgtgctagacagtttaccaggatccgtgggaggtctatcgccatctcaggcatccagcgccgcatcctcggcttcctcaagcccgggttcagggatctccgaagcactcagagctggagcaggttccggcactggatacaacaaggaattcctgctctacctggcgggcttcgtcgacggggacggctccatctttgcctgtatccgtccgtcgcagagggctaagttcaagcacgtgctgcagctccatttccgggtctttcagaagacacagcgccgttggttcctcgacaagctggtggacgagatcggtgtaggttacgtgtatgaccacggcagggcgagcatctaccagctgtcccagatcaagcctctgcacaacttcctgacccagctccagcccttcctgaagctcaagcagaagcaggccaacctcgtgctgaagatcatcgagcagctgccctccgccaaggaatccccggacaagttcctggaggtgtgcacctgggtggaccagatcgccgctctgaacgactcccacacccgcaagaccacttccgaaaccgtccgcgccgttctagacagtctctccgagaagaagaagtcgtccccctaa

SEQ ID NO: 82 - DNA, 1065 bp, Artificial Sequence
  Synthesized
atgaatacaaaatataataaagagttcttactctacttagcagggtttgtagactctgacggttccatcgttgccaggatcgagccggctcaggattgtaagttcaagcacaggctgaggctccagttctttgtctctcagaagacacagcgccgttggttcctcgacaagctggtggacgagatcggtgtgggttacgtgcgggactctggcagcgtctccagttacttgctgtcccagatcaagcctttgcataattttttaacacaactacaaccttttctaaaactaaaacaaaaacaagcaaatttagttttaaaaattattgaacaacttccgtcagcaaaagaatccccggacaaattcttagaagtttgtacatgggtggatcaaattgcagctctgaatgattcgaagacgcgtaaaacaacttctgaaaccgttcgtgctgtgctagacagtttaccaggatccgtgggaggtctatcgccatctcaggcatccagcgccgcatcctcggcttcctcaagcccgggttcagggatctccgaagcactcagagctggagcaggttccggcactggatacaacaaggaattcctgctctacctggcgggcttcgtcgacggggacggctccatctttgcctgtatccgtccgtcgcagagggctaagttcaagcacgtgctgcagctctgtttccgggtctttcagaagacacagcgccgttggttcctcgacaagctggtggacgagatcggtgtaggttacgtgtatgaccacggcagggcgagcatctaccagctgtcccagatcaagcctctgcacaacttcctgacccagctccagcccttcctgaagctcaagcagaagcaggccaacctcgtgctgaagatcatcgagcagctgccctccgccaaggaatccccggacaagttcctggaggtgtgcacctgggtggaccagatcgccgctctgaacgactcccacacccgcaagaccacttccgaaaccgtccgcgccgttctagacagtctctccgagaagaagaagtcgtccccctaa

SEQ ID NO: 83 - DNA, 1065 bp, Artificial Sequence
  Synthesized
atgaatacaaaatataataaagagttcttactctacttagcagggtttgtagacgctgacggttccatcgttgccaggatcgagccggctcaggattgtaagttcaagcacaggctgaggctccagttctttgtctctcagaagacacagcgccgttggttcctcgacaagctggtggacgagatcggtgtgggttacgtgcgggactctggcagcgtctccagttacaatctgtccgagatcaagcctttgcataattttttaacacaactacaaccttttctaaaactaaaacaaaaacaagcaaatttagttttaaaaattattgaacaacttccgtcagcaaaagaatccccggacaaattcttagaagtttgtacatgggtggatcaaattgcagctctgaatgattcgaagacgcgtaaaacaacttctgaaaccgttcgtgctgtgctagacagtttaccaggatccgtgggaggtctatcgccatctcaggcatccagcgccgcatcctcggcttcctcaagcccgggttcagggatctccgaagcactcagagctggagcaggttccggcactggatacaacaaggaattcctgctctacctggcgggcttcgtcgacggggacggctccatctttgcctgtatccgtccgtcgcagagggctaagttcaagcacgtgctgcagctctgtttccgggtctttcagaagacacagcgccgttggttcctcgacaagctggtggacgagatcggtgtaggttacgtgtatgaccacggcagggcgagcatctaccagctgtcccagatcaagcctctgcacaacttcctgacccagctccagcccttcctgaagctcaagcagaagcaggccaacctcgtgctgaagatcatcgagcagctgccctccgccaaggaatccccggacaagttcctggaggtgtgcacctgggtggaccagatcgccgctctgaacgactcccacacccgcaagaccacttccgaaaccgtccgcgccgttctagacagtctctccgagaagaagaagtcgtccccctaa

SEQ ID NO: 84 - protein, 147 aa, Artificial Sequence
  Synthesized
KEFLLYLAGFVDSDGSIYATIRPVQSTKFKHTLRLWFAVTQKTQRRWFLDKLVDEIGVGYVYDNGSVSWYYLSEIKPLHNFLTQLQPFLKLKQKQANLVLKIIEQLPSAKESPDKFLEVCTWVDQIAALNDSKTRKTTSETVRAVLD

SEQ ID NO: 85 - protein, 147 aa, Artificial Sequence
  Synthesized
KEFLLYLAGFVDSDGSIFAVIEPVQSAKFKHRLKLSFVVTQKTQRRWFLDKLVDEIGVGYVYDQGSVSFYRLSEIKPLHNFLTQLQPFLKLKQKQANLVLKIIEQLPSAKESPDKFLEVCTWVDQIAALNDSKTRKTTSETVRAVLD

SEQ ID NO: 86 - protein, 147 aa, Artificial Sequence
  Synthesized
KEFLLYLAGFVDSDGSIYASIMPIQTAKFKHRLKLQFAVAQKTQRRWFLDKLVDEIGVGYVYDFGSVSYYRLSQIKPLHNFLTQLQPFLKLKQKQANLVLKIIEQLPSAKESPDKFLEVCTWVDQIAALNDSKTRKTTSETVRAVLD

SEQ ID NO: 87 - protein, 147 aa, Artificial Sequence
  Synthesized
KEFLLYLAGFVDSDGSIIAFIMPSQTAKFKHRLKLQFAVAQKTQRRWFLDKLVDEIGVGYVYDFGSVSYYRLSQIKPLHNFLTQLQPFLKLKQKQANLVLKIIEQLPSAKESPDKFLEVCTWVDQIAALNDSKTRKTTSETVRAVLD

SEQ ID NO: 88 - protein, 147 aa, Artificial Sequence
  Synthesized
KEFLLYLAGFVDSDGSIMAFIMPTQTAKFKHRLKLQFAVAQKTQRRWFLDKLVDEIGVGYVYDFGSVSYYRLSEIKPLHNFLTQLQPFLKLKQKQANLVLKIIEQLPSAKESPDKFLEVCTWVDQIAALNDSKTRKTTSETVRAVLD

SEQ ID NO: 89 - protein, 147 aa, Artificial Sequence
  Synthesized
KEFLLYLAGFVDSDGSIMAFILPEQHMKFKHRLRLQFAVAQKTQRRWFLDKLVDEIGVGYVYDFGSVSYYRLSEIKPLHNFLTQLQPFLKLKQKQANLVLKIIEQLPSAKESPDKFLEVCTWVDQIAALNDSKTRKTTSETVRAVLD

SEQ ID NO: 90 - protein, 147 aa, Artificial Sequence
  Synthesized
KEFLLYLAGFVDSDGSIMAFILPEQHLKFKHRLRLQFAVAQKTQRRWFLDKLVDEIGVGYVYDFGSVSYYRLSEIKPLHNFLTQLQPFLKLKQKQANLVLKIIEQLPSAKESPDKFLEVCTWVDQIAALNDSKTRKTTSETVRAVLD

SEQ ID NO: 91 - protein, 147 aa, Artificial Sequence
  Synthesized
KEFLLYLAGFVDSDGSIMAFILPEQGLKFKHRLRLQFAVAQKTQRRWFLDKLVDEIGVGYVYDFGSVSYYRLSQIKPLHNFLTQLQPFLKLKQKQANLVLKIIEQLPSAKESPDKFLEVCTWVDQIAALNDSKTRKTTSETVRAVLD

SEQ ID NO: 92 - protein, 147 aa, Artificial Sequence
  Synthesized
KEFLLYLAGFVDSDGSIMAFIMPDQAPKFKHRLRLQFAVAQKTQRRWFLDKLVDEIGVGYVYDFGSVSYYRLSEIKPLHNFLTQLQPFLKLKQKQANLVLKIIEQLPSAKESPDKFLEVCTWVDQIAALNDSKTRKTTSETVRAVLD

SEQ ID NO: 93 - protein, 147 aa, Artificial Sequence
  Synthesized
KEFLLYLAGFVDADGSIYACIKPHQQLKFKHQLLLYFEVYQKTQRRWFLDKLVDEIGVGYVADRGSVSEYRLSQIKPLHNFLTQLQPFLKLKQKQANLVLKIIEQLPSAKESPDKFLEVCTWVDQIAALNDSKTRKTTSETVRAVLD

SEQ ID NO: 94 - protein, 147 aa, Artificial Sequence
  Synthesized
KEFLLYLAGFVDADGSIYACIKPHQQLKFKHQLLLYFEVYQKTQRRWFLDKLVDEIGVGYVIDSGSVSTYRLSQIKPLHNFLTQLQPFLKLKQKQANLVLKIIEQLPSAKESPDKFLEVCTWVDQIAALNDSKTRKTTSETVRAVLD

SEQ ID NO: 95 - protein, 147 aa, Artificial Sequence; identical to SEQ ID NO: 93
  Synthesized

SEQ ID NO: 96 - protein, 147 aa, Artificial Sequence
  Synthesized
KEFLLYLAGFVDSDGSIYACIKPHQQLKFKHQLLLYFEVYQKTQRRWFLDKLVDEIGVGYVADRGSVSEYRLSQIKPLHNFLTQLQPFLKLKQKQANLVLKIIEQLPSAKESPDKFLEVCTWVDQIAALNDSKTRKTTSETVRAVLD

SEQ ID NO: 97 - protein, 147 aa, Artificial Sequence; identical to SEQ ID NO: 93
  Synthesized

SEQ ID NO: 98 - protein, 147 aa, Artificial Sequence; identical to SEQ ID NO: 93
  Synthesized

SEQ ID NO: 99 - protein, 147 aa, Artificial Sequence; identical to SEQ ID NO: 96
  Synthesized

SEQ ID NO: 100 - protein, 147 aa, Artificial Sequence
  Synthesized
KEFLLYLAGFVDADGSIYACIKPHQELKFKHQLLLYFEVYQKTQRRWFLDKLVDEIGVGYVADRGSVSEYRLSEIKPLHNFLTQLQPFLKLKQKQANLVLKIIEQLPSAKESPDKFLEVCTWVDQIAALNDSKTRKTTSETVRAVLD

SEQ ID NO: 101 - protein, 147 aa, Artificial Sequence
  Synthesized
KEFLLYLAGFVDSDGSIVATIRPGQELKFKHGLRLRFYVCQKTQRRWFLDKLVDEIGVGYVTDSGSVSRYELSQIKPLHNFLTQLQPFLKLKQKQANLVLKIIEQLPSAKESPDKFLEVCTWVDQIAALNDSKTRKTTSETVRAVLD

SEQ ID NO: 102 - protein, 147 aa, Artificial Sequence
  Synthesized
KEFLLYLAGFVDADGSIVATIRPGQELKFKHGLRLRFYVCQKTQRRWFLDKLVDEIGAGYVTDSGSVSRYELSQIKPLHNFLTQLQPFLKLKQKQANLVLKIIEQLPSAKESPDKFLEVCTWVDQIAALNDSKTRKTTSETVRAVLD

SEQ ID NO: 103 - protein, 147 aa, Artificial Sequence
  Synthesized
KEFLLYLAGFVDADGSIVATIRPGQELKFKHGLRLRFYVCQKTQRRWFLDKLVDEIGVGYVTDSGSVSRYELSQIKPLHNFLTQLQPFLKLKQKQANLVLKIIEQLPSAKESPDKFLEVCTWVDQIAALNDSKTRKTTSETVRAVLD

SEQ ID NO: 104 - protein, 147 aa, Artificial Sequence
  Synthesized
KEFLLYLAGFVDSDGSIVASIAPAQDCKFKHRLRLRFFVSQKTQRRWFLDKLVDEIGVGYVSDSGSVSSYVLSEIKPLHNFLTQLQPFLKLKQKQANLVLKIIEQLPSAKESPDKFLEVCTWVDQIAALNDSKTRKTTSETVRAVLD

SEQ ID NO: 105 - protein, 147 aa, Artificial Sequence
  Synthesized
KEFLLYLAGFVDSDGSIVARIEPAQDCKFKHRLRLQFFVSQKTQRRWFLDKLVDEIGVGYVRDSGSVSSYDLSQIKPLHNFLTQLQPFLKLKQKQANLVLKIIEQLPSAKESPDKFLEVCTWVDQIAALNDSKTRKTTSETVRAVLD

SEQ ID NO: 106 - protein, 147 aa, Artificial Sequence
  Synthesized
KEFLLYLAGFVDSDGSIVARIEPAQDCKFKHRLRLQFFVSQKTQRRWFLDKLVDEIGVGYVRDSGSVSSYLLSQIKPLHNFLTQLQPFLKLKQKQANLVLKIIEQLPSAKESPDKFLEVCTWVDQIAALNDSKTRKTTSETVRAVLD

SEQ ID NO: 107 - protein, 147 aa, Artificial Sequence
  Synthesized
KEFLLYLAGFVDADGSIVARIEPAQDCKFKHRLRLQFFVSQKTQRRWFLDKLVDEIGVGYVRDSGSVSSYNLSEIKPLHNFLTQLQPFLKLKQKQANLVLKIIEQLPSAKESPDKFLEVCTWVDQIAALNDSKTRKTTSETVRAVLD

SEQ ID NO: 108 - protein, 147 aa, Artificial Sequence
  Synthesized
KEFLLYLAGFVDGDGSICACIVPRQDRKFKHQLRLFFEVGQKTKRRWFLDKLVDEIGVGYVEDTGRASRYRLSQIKPLHNFLTQLQPFLKLKQKQANLVLKIIEQLPSAKESPDKFLEVCTWVDQIAALNDSRTRKTTSETVRAVLD

SEQ ID NO: 109 - protein, 147 aa, Artificial Sequence
  Synthesized
KEFLLYLAGFVDGDGSICACIVPRQDRKFKHQLRLFFEVGQTTRRRWFLDKLVDEIGVGYVFDKGSASMYRLSEIKPLHNFLTQLQPFLKLKQKQANLVLKIIEQLPSAKESPDKFLEVCTWVDQIAALNDSRTRKTTSETVRAVLD

SEQ ID NO: 110 - protein, 147 aa, Artificial Sequence
  Synthesized
KEFLLYLAGFVDGDGSICACIVPRQDRKFKHQLRLFFEVGQKTQRRWFLDKLVDEIGVGYVRDLGSASTYRLSEIKPLHNFLTQLQPFLKLKQKQANLVLKIIEQLPSAKESPDKFLEVCTWVDQIAALNDSRTRKTTSETVRAVLD

SEQ ID NO: 111 - protein, 147 aa, Artificial Sequence
  Synthesized
KEFLLYLAGFVDGDGSICACIVPRQDRKFKHQLRLFFEIGQKTQRRWFLDKLVDEIGVGYVRDLGSASTYRLSQIKPLHNFLTQLQPFLKLKQKQANLVLKIIEQLPSAKESPDKFLEVCTWVDQIAALNDSKTRKTTSETVRAVLD

SEQ ID NO: 112 - protein, 147 aa, Artificial Sequence
  Synthesized
KEFLLYLAGFVDGDGSICACIVPRQDRKFKHQLRLFFEVGQKTQRRWFLDKLVDEIGVGYVRDLGSASTYRLSQIKPLHNFLTQLQPFLKLKQKQANLVLKIIEQLPSAKESPDKFLEVCTWVDQIAALNDSRTRKTTSETVRAVLD

SEQ ID NO: 113 - protein, 147 aa, Artificial Sequence; identical to SEQ ID NO: 110
  Synthesized

SEQ ID NO: 114 - protein, 147 aa, Artificial Sequence; identical to SEQ ID NO: 110
  Synthesized

SEQ ID NO: 115 - protein, 147 aa, Artificial Sequence; identical to SEQ ID NO: 112
  Synthesized

SEQ ID NO: 116 - protein, 147 aa, Artificial Sequence; identical to SEQ ID NO: 112
  Synthesized

SEQ ID NO: 117 - protein, 147 aa, Artificial Sequence
  Synthesized
KEFLLYLAGFVDGDGSIFASIMPTQWTKFKHSLLLRFRVTQSTRRRWFLDKLMDEIGVGYVSDQGRASYYTLSEIKPLHNFLTQLQPFLKLKQKQANLVLKIIEQLPSAKESPDKFLEVCTWVDQIAALNDSRTRKTTSETVRAVLD

SEQ ID NO: 118 - protein, 147 aa, Artificial Sequence
  Synthesized
KEFLLYLAGFVDGDGSIFASIIPSQLVKFKHTLLLRFRVTQATRRRWFLDKLVDEIGVGYVTDNGRASYYTLSEIKPLHNFLTQLQPFLKLKQKQANLVLKIIEQLPSAKESPDKFLEVCTWVDQIAALNDSRTRKTTSETVRAVLD

SEQ ID NO: 119 - protein, 147 aa, Artificial Sequence
  Synthesized
KEFLLYLAGFVDGDGSIFASIIPSQLVKFKHTLLLRFRVCQATKRRWFLDKLVDEIGVGYVSDQGSASYYTLSEIKPLHNFLTQLQPFLKLKQKQANLVLKIIEQLPSAKESPDKFLEVCTWVDQIAALNDSRTRKTTSETVRAVLD

SEQ ID NO: 120 - protein, 147 aa, Artificial Sequence
  Synthesized
KEFLLYLAGFVDGDGSIFASIIPSQEVKFKHTLLLRFRVCQATKRRWFLDKLVDEIGVGYVSDQGSASYYTLSEIKPLHNFLTQLQPFLKLKQKQANLVLKIIEQLPSAKESPDKFLEVCTWVDQIAALNDSRTRKTTSETVRAVLD

SEQ ID NO: 121 - protein, 147 aa, Artificial Sequence; identical to SEQ ID NO: 120
  Synthesized

SEQ ID NO: 122 - protein, 147 aa, Artificial Sequence
  Synthesized
KEFLLYLAGFVDGDGSIFASIIPSQEVKFKHTLLLRFRVTQATKRRWFLDKLVDEIGVGYVSDVGSASYYTLSEIKPLHNFLTQLQPFLKLKQKQANLVLKIIEQLPSAKESPDKFLEVCTWVDQIAALNDSRTRKTTSETVRAVLD

SEQ ID NO: 123 - protein, 147 aa, Artificial Sequence
  Synthesized
KEFLLYLAGFVDGDGSIFASIIPSQEVKFKHTLLLRFRVCQATKRRWFLDKLVDEIGVGYVSDRGSASYYTLSEIKPLHNFLTQLQPFLKLKQKQANLVLKIIEQLPSAKESPDKFLEVCTWVDQIAALNDSRTRKTTSETVRAVLD

SEQ ID NO: 124 - protein, 147 aa, Artificial Sequence
  Synthesized
KEFLLYLAGFVDGDGSIFASIIPSQEVKFKHTLLLRFRVCQATKRRWFLDKLVDEIGVGYVSDQGSASYYTLSQIKPLHNFLTQLQPFLKLKQKQANLVLKIIEQLPSAKESPDKFLEVCTWVDQIAALNDSRTRKTTSETVRAVLD

SEQ ID NO: 125 - protein, 147 aa, Artificial Sequence
  Synthesized
KEFLLYLAGFVDGDGSIFACIRPSQRAKFKHVLQLCFRVHQLTKRRWFLDKLVDEIGVGYVYDCGSASFYHLSQIKPLHNFLTQLQPFLKLKQKQANLVLKIIEQLPSAKESPDKFLEVCTWVDQIAALNDSKTRKTTSETVRAVLD

SEQ ID NO: 126 - protein, 147 aa, Artificial Sequence
  Synthesized
KEFLLYLAGFVDGDGSIFACIRPSQRAKFKHVLQLCFRVHQKTKRRWFLDKLVDEIGVGYVYDHGSASCYHLSEIKPLHNFLTQLQPFLKLKQKQANLVLKIIEQLPSAKESPDKFLEVCTWVDQIAALNDSHTRKTTSETVRAVLD

SEQ ID NO: 127 - protein, 147 aa, Artificial Sequence
  Synthesized
KEFLLYLAGFVDGDGSIFACIRPSQRAKFKHVLQLCFRVHQSTRRRWFLDKLVDEIGAGYVYDHGSASLYSLSQIKPLHNFLTQLQPFLKLKQKQANLVLKIIEQLPSAKESPDKFLEVCTWVDQIAALNDSHTRKTTSETVRAVLD

SEQ ID NO: 128 - protein, 147 aa, Artificial Sequence
  Synthesized
KEFLLYLAGFVDGDGSIFACIRPSQRAKFKHVLQLCFRVFQKTQRRWFLDKLVDEIGVGYVYDHGRASIYQLSQIKPLHNFLTQLQPFLKLKQKQANLVLKIIEQLPSAKESPDKFLEVCTWVDQIAALNDSHTRKTTSETVRAVLD

SEQ ID NO: 129 - protein, 147 aa, Artificial Sequence
  Synthesized
KEFLLYLAGFVDGDGSIFACIRPSQRAKFKHVLQLHFRVFQKTQRRWFLDKLVDEIGVGYVYDHGRASIYQLSQIKPLHNFLTQLQPFLKLKQKQANLVLKIIEQLPSAKESPDKFLEVCTWVDQIAALNDSHTRKTTSETVRAVLD

SEQ ID NO: 130 - protein, 147 aa, Artificial Sequence; identical to SEQ ID NO: 128
  Synthesized

SEQ ID NO: 131 - protein, 147 aa, Artificial Sequence; identical to SEQ ID NO: 128
  Synthesized

SEQ ID NO: 132 - protein, 42 aa, Artificial Sequence
  Synthesized
SLPGSVGGLSPSQASSAASSASSSPGSGISEALRAGAGSGTG

SEQ ID NO: 133 - DNA, 20 bp, Artificial Sequence
  Synthesized
cgggaggtaatacataatcc

SEQ ID NO: 134 - DNA, 21 bp, Artificial Sequence
  Synthesized
gggtgggttgctttacctctc

SEQ ID NO: 135 - DNA, 20 bp, Artificial Sequence
  Synthesized
tgggctactgcaactctgtt

SEQ ID NO: 136 - DNA, 27 bp, Artificial Sequence
  Synthesized
aggacaaaagaggacggtctgccctgg

SEQ ID NO: 137 - DNA, 20 bp, Artificial Sequence
  Synthesized
taagacccagcttcacggag

SEQ ID NO: 138 - DNA, 20 bp, Artificial Sequence
  Synthesized
tatgatcgcctgttcctcca

SEQ ID NO: 139 - DNA, 18 bp, Artificial Sequence
  Synthesized
ctggccgaagtataggaa

SEQ ID NO: 140 - DNA, 21 bp, Artificial Sequence
  Synthesized
cgcaacatgtgacataaagag

SEQ ID NO: 141 - DNA, 20 bp, Artificial Sequence
  Synthesized
tctggatatcctcttctggg

SEQ ID NO: 142 - DNA, 19 bp, Artificial Sequence
  Synthesized
cctacatggtgtatctgac

SEQ ID NO: 143 - DNA, 21 bp, Artificial Sequence
  Synthesized
gaacaccaccagaaaaacaag

SEQ ID NO: 144 - DNA, 21 bp, Artificial Sequence
  Synthesized
cacttcctgtaagacaaccag

SEQ ID NO: 145 - DNA, 17 bp, Artificial Sequence
  Synthesized
atccctcatacccaatc

SEQ ID NO: 146 - DNA, 20 bp, Artificial Sequence
  Synthesized
aaaaaccacggtgctgttga

SEQ ID NO: 147 - DNA, 20 bp, Artificial Sequence
  Synthesized
atggggtccgagacttttcc

SEQ ID NO: 148 - DNA, 21 bp, Artificial Sequence
  Synthesized
gggtgggttgctttacctctc

SEQ ID NO: 149 - DNA, 19 bp, Artificial Sequence
  Synthesized
agagcatgccatctgagtc

SEQ ID NO: 150 - DNA, 20 bp, Artificial Sequence
  Synthesized
gtgaagtagcaaagcacctg

SEQ ID NO: 151 - DNA, 19 bp, Artificial Sequence
  Synthesized
agagcatgccatctgagtc

SEQ ID NO: 152 - DNA, 21 bp, Artificial Sequence
  Synthesized
gggtgggttgctttacctctc

SEQ ID NO: 153 - DNA, 20 bp, Artificial Sequence
  Synthesized
tttggtatggggtccgagac

SEQ ID NO: 154 - DNA, 20 bp, Artificial Sequence
  Synthesized
gtgaagtagcaaagcacctg

SEQ ID NO: 155 - DNA, 20 bp, Artificial Sequence
  Synthesized
tttggtatggggtccgagac

SEQ ID NO: 156 - DNA, 21 bp, Artificial Sequence
  Synthesized
gggtgggttgctttacctctc

SEQ ID NO: 157 - DNA, 23 bp, Artificial Sequence
  Synthesized
gattctcagaaatggagtgactg

SEQ ID NO: 158 - DNA, 20 bp, Artificial Sequence
  Synthesized
gtgaagtagcaaagcacctg

SEQ ID NO: 159 - DNA, 23 bp, Artificial Sequence
  Synthesized
gattctcagaaatggagtgactg

SEQ ID NO: 160 - DNA, 25 bp, Artificial Sequence
  Synthesized
atcagaaggattatgtataggaata

SEQ ID NO: 161 - DNA, 20 bp, Artificial Sequence
  Synthesized
gggtgggttgctttacctct

SEQ ID NO: 162 - DNA, 20 bp, Artificial Sequence
  Synthesized
tctggatatcctcttctggg

SEQ ID NO: 163 - DNA, 20 bp, Artificial Sequence
  Synthesized
gtgaagtagcaaagcacctg

SEQ ID NO: 164 - DNA, 20 bp, Artificial Sequence
  Synthesized
gtgaagtagcaaagcacctg

SEQ ID NO: 165 - DNA, 25 bp, Artificial Sequence
  Synthesized
agtcacttcctaagctaagacaacc

SEQ ID NO: 166 - DNA, 24 bp, Artificial Sequence
  Synthesized
cagaaggattatgtatgagggata

SEQ ID NO: 167 - DNA, 20 bp, Artificial Sequence
  Synthesized
gtgaagtagcaaagcacctg

SEQ ID NO: 168 - DNA, 20 bp, Artificial Sequence
  Synthesized
atggggtccgagacttttcc

SEQ ID NO: 169 - DNA, 335 bp, Artificial Sequence
  Synthesized
cggccgtccgccttcggcaccatcctcacgacacccaaatatggcgacgggtgaggaatggtggggagttatttttagagcggtgaggaaggtgggcaggcagcaggtgttggcgctctaaaaataactcccgggagttatttttagagcggaggaatggtggacacccaaatatggcgacggttcctcacccgtcgccatatttgggtgtccgccctcggccggggccgcattcctgggggccgggcggtgctcccgcccgcctcgataaaaggctccggggccggcggcggcccacgagctacccggaggagcgggaggcgccaagctctaga

SEQ ID NO: 170 - DNA, 3357 bp, Mus Musculus
ccatcctggtctatagagagagttccagaacagccagggctacagataaacccatctggaaaaacaaagttgaatgacccaagaggggttctcagagggtggcgtgtgctccctggcaagcctatgacatggccggggcctgcctctctctgcctctgaccctcagtggctcccatgaactccttgcccaatggcatctttttcctgcgctccttgggttattccagtctcccctcagcattccttcctcagggcctcgctcttctctctgctccctccttgcacagctggctctgtccacctcagatgtcacagtgctctctcagaggaggaaggcaccatgtaccctctgtttcccaggtaagggttcaatttttaaaaatggttttttgtttgtttgtttgtttgtttgtttgtttgtttttcaagacagggctcctctgtgtagtcctaactgtcttgaaactccctctgtagaccaggtcgacctcgaactcttgaaacctgccacggaccacccagtcaggtatggaggtccctggaatgagcgtcctcgaagctaggtgggtaagggttcggcggtgacaaacagaaacaaacacagaggcagtttgaatctgagtgtattttgcagctctcaagcaggggattttatacataaaaaaaaaaaaaaaaaaaaaaccaaacattacatctcttagaaactatatccaatgaaacaatcacagataccaaccaaaaccattgggcagagtaaagcacaaaaatcatccaagcattacaactctgaaaccatgtattcagtgaatcacaaacagaacaggtaacatcattattaatataaatcaccaaaatataacaattctaaaaggatgtatccagtgggggctgtcgtccaaggctagtggcagatttccaggagcaggttagtaaatcttaaccactgaactaactctccagccccatggtcaattattatttagcatctagtgcctaatttttttttataaatcttcactatgtaatttaaaactattttaattcttcctaattaaggctttctttaccatataccaaaattcacctccaatgacacacgcgtagccatatgaaattttattgttgggaaaatttgtacctatcataatagttttgtaaatgatttaaaaagcaaagtgttagccgggcgtggtggcacacgcctttaatccctgcactcgggaggcaggggcaggaggatttctgagtttgaggccagcctggtctacagagtgagttccaggacagccagggctacacagagaaaccctgtctcgaaccccccaccccccaaaaaaagcaaagtgttggtttccttggggataaagtcatgttagtggcccatctctaggcccatctcacccattattctcgcttaagatcttggcctaggctaccaggaacatgtaaataagaaaaggaataagagaaaacaaaacagagagattgccatgagaactacggctcaatattttttctctccggcgaagagttccacaaccatctccaggaggcctccacgttttgaggtcaatggcctcagtctgtggaacttgtcacacagatcttactggaggtggtgtggcagaaacccattccttttagtgtcttgggctaaaagtaaaaggcccagaggaggcctttgctcatctgaccatgctgacaaggaacacgggtgccaggacagaggctggaccccaggaacaccttaaacacttcttcccttctccgccccctagagcaggctcccctcaccagcctgggcagaaatgggggaagatggagtgaagccatactggctactccagaatcaacagagggagccgggggcaatactggagaagctggtctccccccaggggcaatcctggcacctcccaggcagaagaggaaacttccacagtgcatctcacttccatgaatcccctcctcggactctgaggtccttggtcacagctgaggtgcaaaaggctcctgtcatattgtgtcctgctctggtctgccttccacagcttgggggccacctagcccacctctccctagggatgagagcagccactacgggtctaggctgcccatgtaaggaggcaaggcctggggacacccgagatgcctggttataattaacccagacatgtggctgcccccccccccccaacacctgctgcctgagcctcacccccaccccggtgcctgggtcttaggctctgtacaccatggaggagaagctcgctctaaaaataaccctgtccctggtggatccagggtgaggggcaggctgagggcggccacttccctcagccgcaggtttgttttcccaagaatggtttttctgcttctgtagcttttcctgtcaattctgccatggtggagcagcctgcactgggcttctgggagaaaccaaaccgggttctaacctttcagctacagttattgcctttcctgtagatgggcgactacagccccacccccacccccgtctcctgtatccttcctgggcctggggatcctaggctttcactggaaatttccccccaggtgctgtaggctagagtcacggctcccaagaacagtgcttgcctggcatgcatggttctgaacctccaactgcaaaaaatgacacataccttgacccttggaaggctgaggcagggggattgccatgagtgcaaagccagactgggtggcatagttagaccctgtctcaaaaaaccaaaaacaattaaataactaaagtcaggcaagtaatcctactcgggagactgaggcagagggattgttacatgtctgaggccagcctggactacatagggtttcaggctagccctgtctacagagtaaggccctatttcaaaaacacaaacaaaatggttctcccagctgctaatgctcaccaggcaatgaagcctggtgagcattagcaatgaaggcaatgaaggagggtgctggctacaatcaaggctgtgggggactgagggcaggctgtaacaggcttgggggccagggcttatacgtgcctgggactcccaaagtattactgttccatgttcccggcgaagggccagctgtcccccgccagctagactcagcacttagtttaggaaccagtgagcaagtcagcccttggggcagcccatacaaggccatggggctgggcaagctgcacgcctgggtccggggtgggcacggtgcccgggcaacgagctgaaagctcatctgctctcaggggcccctccctggggacagcccctcctggctagtcacaccctgtaggctcctctatataacccaggggcacaggggctgcccccgggtcac

SEQ ID NO: 171 - DNA, 655 bp, Homo sapiens
cctgagtttgaatctctccaactcagccagcctcagtttcccctccactcagtccctaggaggaaggggcgcccaagcgggtttctggggttagactgccctccattgcaattggtccttctcccggcctctgcttcctccagctcacagggtatctgctcctcctggagccacaccttggttccccgaggtgccgctgggactcgggtaggggtgagggcccaggggcgacagggggagccgagggccacaggaagggctggtggctgaaggagactcaggggccaggggacggtggcttctacgtgcttgggacgttcccagccaccgtcccatgttcccggcgggggccagctgtccccaccgccagcccaactcagcacttggttagggtatcagcttggtgggggcgtgagcccagccctggggcgctcagcccatacaaggccatggggctgggcgcaaagcatgcctgggttcagggtgggtatggtgccggagcagggaggtgagaggctcagctgccctccagaactcctccctggggacaacccctcccagccaatagcacagcctaggtccccctatataaggccacggctgctggcccttcctttgggtcagtgtcacctccaggatacagacagcccccctt

SEQ ID NO: 172 - DNA, 206 bp, Mus Musculus
ccactacgggtctaggctgcccatgtaaggaggcaaggcctggggacacccgagatgcctggttataattaacccagacatgtggctgcccccccccccccaacacctgctgcctgagcctcacccccaccccggtgcctgggtcttaggctctgtacaccatggaggagaagctcgctctaaaaataaccctgtccctggtggat

SEQ ID NO: 173 - DNA, 211 bp, Artificial Sequence
  Synthesized
ccactacgggtctaggctgcccatgtaaggaggcaaggcctggggacacccgagatgcctggttataattaaccccaacacctgctgcccccccccccccaacacctgctgcctgagcctgagcggttaccccaccccggtgcctgggtcttaggctctgtacaccatggaggagaagctcgctctaaaaataaccctgtccctggtggat

SEQ ID NO: 174 - DNA, 334 bp, Artificial Sequence
  Synthesized
tggccaccgccttcggcaccatcctcacgacacccaaatatggcgacgggtgaggaatggtggggagttatttttagagcggtgaggaaggtgggcaggcagcaggtgttggcgctctaaaaataactcccgggagttatttttagagcggaggaatggtggacacccaaatatggcgacggttcctcacccgtcgccatatttgggtgtccgccctcggccggggccgcattcctgggggccgggcggtgctcccgcccgcctcgataaaaggctccggggccggcggcggcccacgagctacccggaggagcgggaggcgccaagctctaga

SEQ ID NO: 175 - DNA, 792 bp, artificial Sequence
  Synthesized
aagcttgcatgtctaagctagacccttcagattaaaaataactgaggtaagggcctgggtaggggaggtggtgtgagacgctcctgtctctcctctatctgcccatcggccctttggggaggaggaatgtgcccaaggactaaaaaaaggccatggagccagaggggcgagggcaacagacctttcatgggcaaaccttggggccctgctgtctagcatgccccactacgggtctaggctgcccatgtaaggaggcaaggcctggggacacccgagatgcctggttataattaacccagacatgtggctgcccccccccccccaacacctgctgcctctaaaaataaccctgtccctggtggatcccctgcatgcgaagatcttcgaacaaggctgtgggggactgagggcaggctgtaacaggcttgggggccagggcttatacgtgcctgggactcccaaagtattactgttccatgttcccggcgaagggccagctgtcccccgccagctagactcagcacttagtttaggaaccagtgagcaagtcagcccttggggcagcccatacaaggccatggggctgggcaagctgcacgcctgggtccggggtgggcacggtgcccgggcaacgagctgaaagctcatctgctctcaggggcccctccctggggacagcccctcctggctagtcacaccctgtaggctcctctatataacccaggggcacaggggctgccctcattctaccaccacctccacagcacagacagacactcaggagcagccagc

SEQ ID NO: 176 - DNA, 450 bp, artificial Sequence
  Synthesized
ctagactagcatgctgcccatgtaaggaggcaaggcctggggacacccgagatgcctggttataattaacccagacatgtggctgcccccccccccccaacacctgctgcctctaaaaataaccctgcatgccatgttcccggcgaagggccagctgtcccccgccagctagactcagcacttagtttaggaaccagtgagcaagtcagcccttggggcagcccatacaaggccatggggctgggcaagctgcacgcctgggtccggggtgggcacggtgcccgggcaacgagctgaaagctcatctgctctcaggggcccctccctggggacagcccctcctggctagtcacaccctgtaggctcctctatataacccaggggcacaggggctgccctcattctaccaccacctccacagcacagacagacactcaggagccagccagc

SEQ ID NO: 177 - DNA, 1417 bp, Artificial Sequence
  Synthesized
ttctgagtcctctaaggtccctcactcccaactcagccccatgtcctgtcaattcccactcagtgtctgatctccttctcctcacctttcccatctcccgtttgacccagcttcctgagctctcctcccattcccctttttggagtcctcctcctctcccagaacccagtaataagtgggctcctccctggcctggacccccgtggtaaccctataaggcgaggcagctgctgtctgaggcagggaggggctggtgtgggaggctaagggcagctgctaagtttagggtggctccttctctcttcttagagacaacaggtggctggggcctcagtgcccagaaaagaaaatgtcttagaggtatcggcatgggcctggaggaggggggacagggcagggggaggcatcttcctcaggacatcgggtcctagaggaccttgcttcctagctgggcctttccttctcctctataaataccagctctggtatttcgccttggcagctgttgctgctagggagacggctggcttgacatgcatctcctgacaaaacacaaacccgtggtgtgagtgggtgtgggcggtgtgagtagggggatgaatcagagagggggcgagggagacaggggcgcaggagtcaggcaaaggcgatgcgggggtgcgactacacgcagttggaaacagtcgtcagaagattctggaaactatcttgctggctataaacttgagggaagcagaaggccaacattcctcccaagggaaactgaggctcagagttaaaacccaggtatcagtgatatgcatgtgccccggccagggtcactctctgactaaccggtacctaccctacaggcctacctagagactcttttgaaaggatggtagagacctgtccgggctttgcccacagtcgttggaaacctcagcattttctaggcaacttgtgcgaataaaacacttcgggggtccttcttgttcattccaataacctaaaacctctcctcggagaaaatagggggcctcaaacaaacgaaattctctagcccgctttccccaggataaggcaggcatccaaatggaaaaaaaggggccggccgggggtctcctgtcagctccttgccctgtgaaacccagcaggcctgcctgtcttctgtcctcttggggctgtccaggggcgcaggcctcttgcgggggagctggcctccccgccccctcgcctgtggccgcccttttcctggcaggacagagggatcctgcagctgtcaggggaggggcgccggggggtgatgtcaggagggctacaaatagtgcagacagctaaggggctccgtcacccatcttcacatccactccagccggctgcccgcccgctgcctcctctgtgcgtccgcccagccagcctcgtccacgccgccacc

SEQ ID NO: 178 - DNA, 579 bp, Artificial Sequence
  Synthesized
accaacgactgattaactctacgtacgaaacgtatgaagacggacgacccctcggacccctgaaaggtgtggccctcaataaaaatctcgcatatggcgacggcccttggcagtacatcaaaacctttcagggcaatcacgataaccgaccccagccaatagcaccaacgactgattaactctacgtacgaaacgtatgaagacggacgacccctcggacccctgaaaggtgtggcactccttaccacggtccgtatagcccaaactacatgacggttcccagccaatagccgctctaaaaataactcccggcagcggtataaacccacagcgctctaaaaataactcccccggcagcggtatagggcccctccctggggacagccccaacctttcagggcaatcacggtccgcccggtaaatggcaccctcaataaaaatctcgcatccctttggacttcggccccattgacgtcaatggggtccaaaaaatatatcaggggcttcaggtttccctacaaggcctggggacaacccgatatgcctgggtccaaaaaatatatcaggtggttcagtcgt

SEQ ID NO: 179 - DNA, 346 bp, Artificial Sequence
  Synthesized
acaggggtccggaacggcagcggtataaacccacagtggttcagtcgtccgtccgtcgtccacaaccgtccaaaaaatatatcaggaactacatgacggttcaccaacgactgattaactctacgtacgaaacgtatgaagacggacgacccctcggacccctgaaaggtgtggaccaacgactgattaactctacgtacgaaacgtatgaagacggacgacccctcggacccctgaaaggtgtgggtccaaaaaatatatcaggggacacccgagatgcctggttaaactacatgacggttcccccgacaggggtccctccccgggtaataactgcagttacccg

SEQ ID NO: 180 - DNA, 301 bp, Artificial Sequence
  Synthesized
accaacgactgattaactctacgtacgaaacgtatgaagacggacgacccctcggacccctgaaaggtgtggcttggcagtacatcaagcccattgacgtcaataatcttggcagtacatcaaaccaacgactgattaactctacgtacgaaacgtatgaagacggacgacccctcggacccctgaaaggtgtggaccaacgactgattaactctacgtacgaaacgtatgaagacggacgacccctcggacccctgaaaggtgtgggtccaaaaaatatatcaggcaaggcctggggaca

SEQ ID NO: 181 - DNA, 1033 bp, Artificial Sequence
  Synthesized
gcggccgcatcgatattcgtaaacgcgttccttgacacctctgtctcctcaggtgcctggctcccagtccccagaacgcctctcctgtaccttgcttcctagctgggcctttccttctcctctataaataccagctctggtatttcgccttggcagctgttgctgctagggcgcgccgtttaaaccacgtgctcgagagcagccactacgggtctaggctgcccatgtaaggaggcaaggcctggggacacccgagatgcctggttataattaacccagacatgtggctgcccccccccacaacacctgctgcctgagcctcacccccaccccggtgcctgggtcttaggctctgtacaccatggaggagaagctcgctctaaaaataaccctgtcgacacgtgtctagactgatcaatcaaggctgtgggggactgagggcaggctgtaacaggcttgggggccagggcttatacgtgcctgggactcccaaagtattactgttccatgttcccggcgaagggccagctgtcccccgccagctagactcagcacttagtttaggaaccagtgagcaagtcagcccttggggcagcccatacaaggccatggggctgggcaagctgcacgcctgggtccggggtgggcacggtgcccgggcaacgagctgaaagctcatctgctctcaggggcccctccctggggacagcccctcctggctgatcacaccctgtaggctcctctatataacccaggggcactagtgggctgccctcagttcaccaccacctccacagcacagacagacactcaggagccagccaggtacccaggtagggactggccaccccagcccacctgtcccaatgctgacttagtgcaaggcgagccagcaaggagggaggacaggtggcagtggggggtgaggagcatctaaaaatagccacaaactgagttcttaagtctgaacccggtctgctcgcaggtaccggtcccaaaggccgccaccgctagcgatatcggatcctcatga

SEQ ID NO: 182 - protein, 738 aa, Artificial Sequence
  Synthesized
MAADGYLPDWLEDNLSEGIREWWDLKPGAPKPKANQQKQDNGRGLVLPGYKYLGPFNGLDKGEPVNAADAAALEHDKAYDQQLQAGDNPYLRYNHADAEFQERLQEDTSFGGNLGRAVFQAKKRVLEPLGLVESPVKTAPGKKRPVEPSPQRSPDSSTGIGKKGQQPAKKRLNFGQTGDSESVPDPQPIGEPPAGPSGLGSGTMAAGGGAPMADNNEGADGVGSSSGNWHCDSTWLGDRVITTSTRTWALPTYNNHLYKQISNGTSGGSTNDNTYFGYSTPWGYFDFNRFHCHFSPRDWQRLINNNWGFRPKRLNFKLFNIQVKEVTQNEGTKTIANNLTSTIQVFTDSEYQLPYVLGSAHQGCLPPFPADVFMIPQYGYLTLNNGSQAVGRSSFYCLEYFPSQMLRTGNNFEFSYNFEDVPFHSSYAHSQSLDRLMNPLIDQYLYYLSRTQSTGGTAGTQQLLFSQAGPNNMSAQAKNWLPGPCYRQQRVSTTLSQNNNSNFAWTGATKYHLNGRDSLVNPGVAMATHKDDEERFFPSSGVLMFGKQGAGKDNVDYSSVMLTSEEEIKTTNPVATEQYGVVADNLQQQNAAPIVGAVNSQGALPGMVWQNRDVYLQGPIWAKIPHTDGNFHPSPLMGGFGLKHPPPQILIKNTPVPADPPTTFNQAKLASFITQYSTGQVSVEIEWELQKENSKRWNPEIQYTSNYYKSTNVDFAVNTEGTYSEPRPIGTRYLTRNL

SEQ ID NO: 183 - protein, 736 aa, Artificial Sequence
  Synthesized
MAADGYLPDWLEDNLSEGIREWWALKPGAPQPKANQQHQDNARGLVLPGYKYLGPGNGLDKGEPVNAADAAALEHDKAYDQQLKAGDNPYLKYNHADAEFQERLKEDTSFGGNLGRAVFQAKKRLLEPLGLVEEAAKTAPGKKRPVEQSPQEPDSSAGIGKSGAQPAKKRLNFGQTGDTESVPDPQPIGEPPAAPSGVGSLTMASGGGAPVADNNEGADGVGSSSGNWHCDSQWLGDRVITTSTRTWALPTYNNHLYKQISNSTSGGSSNDNAYFGYSTPWGYFDFNRFHCHFSPRDWQRLINNNWGFRPKRLNFKLFNIQVKEVTDNNGVKTIANNLTSTVQVFTDSDYQLPYVLGSAHEGCLPPFPADVFMIPQYGYLTLNDGSQAVGRSSFYCLEYFPSQMLRTGNNFQFSYEFENVPFHSSYAHSQSLDRLMNPLIDQYLYYLSKTINGSGQNQQTLKFSVAGPSNMAVQGRNYIPGPSYRQQRVSTTVTQNNNSEFAWPGASSWALNGRNSLMNPGPAMASHKEGEDRFFPLSGSLIFGKQGTGRDNVDADKVMITNEEEIKTTNPVATESYGQVATNHQSAQAQAQTGWVQNQGILPGMVWQDRDVYLQGPIWAKIPHTDGNFHPSPLMGGFGMKHPPPQILIKNTPVPADPPTAFNKDKLNSFITQYSTGQVSVEIEWELQKENSKRWNPEIQYTSNYYKSNNVEFAVNTEGVYSEPRPIGTRYLTRNL

SEQ ID NO: 184 - DNA, 24 bp, Artificial Sequence
  Synthesized
gctgaacagtttctcagaaagaca

SEQ ID NO: 185 - DNA, 22 bp, Artificial Sequence
  Synthesized
ggctgttttcatccaggttgtg

SEQ ID NO: 186 - DNA, 18 bp, Artificial Sequence
  Synthesized
tcttaaggacctccaagg

SEQ ID NO: 187 - DNA, 24 bp, Artificial Sequence
  Synthesized
gggtgggttgctttacctctctag

SEQ ID NO: 188 - DNA, 26 bp, Artificial Sequence
  Synthesized
tcacatcatgagatttagtcacttcc

SEQ ID NO: 189 - DNA, 25 bp, Artificial Sequence
  Synthesized
ttgctacttcacagtaaccacatgg

SEQ ID NO: 190 - DNA, 20 bp, Artificial Sequence
  Synthesized
gggtgggttgctttacctct

SEQ ID NO: 191 - DNA, 20 bp, Artificial Sequence
  Synthesized
tctggatatcctcttctggg

SEQ ID NO: 192 - DNA, 25 bp, Artificial Sequence
  Synthesized
atcagaaggattatgtataggaata